European Patent Application EP 4 245 376 A2, published September 20, 2023. Title: ANTIBODY MOLECULES TO PD-L1 AND USES THEREOF. Applicant: NOVARTIS AG. The sequence listing filed with the application follows.

SEQUENCE LISTING (362 sequences)

SEQ ID NO: 1 - protein, 5 aa, synthetic construct
  REGION 1..5: note = source = /note="Description of Artificial Sequence: Synthetic peptide"
SYWMY

SEQ ID NO: 2 - protein, 17 aa, synthetic construct
  REGION 1..17: note = source = /note="Description of Artificial Sequence: Synthetic peptide"
RIDPNSGSTKYNEKFKN

SEQ ID NO: 3 - protein, 11 aa, synthetic construct
  REGION 1..11: note = source = /note="Description of Artificial Sequence: Synthetic peptide"
DYRKGLYAMDY

SEQ ID NO: 4 - protein, 7 aa, synthetic construct
  REGION 1..7: note = source = /note="Description of Artificial Sequence: Synthetic peptide"
GYTFTSY

SEQ ID NO: 5 - protein, 6 aa, synthetic construct
  REGION 1..6: note = source = /note="Description of Artificial Sequence: Synthetic peptide"
DPNSGS

SEQ ID NO: 6 - protein, 120 aa, synthetic construct
  REGION 1..120: note = source = /note="Description of Artificial Sequence: Synthetic polypeptide"
QVHLQQPGAELVKPGASVKLSCKASGYTFTSYWMYWVKQGPGRGLEWIGRIDPNSGSTKYNEKFKNKATLTVDKSSSTAYMQLSSLTSEDSAVYYCARDYRKGLYAMDYWGQGTSVTVSS

SEQ ID NO: 7 - DNA, 360 bp, synthetic construct
  misc_feature 1..360: note = source = /note="Description of Artificial Sequence: Synthetic polynucleotide"
  source 1..360: mol_type = other DNA
caggtccacctgcagcagcctggggctgagcttgtgaagcctggggcttcagtgaagctgtcctgcaaggcttctggctacaccttcaccagttactggatgtactgggtgaaacaggggcctggacgaggccttgagtggattggaaggattgatcctaatagtgggagtactaagtacaatgagaagttcaagaacaaggccacactgactgtagacaaatcctccagcacagcctacatgcagctcagcagcctgacatctgaggactctgcggtctattattgtgcaagggactatagaaaggggctctatgctatggactactggggtcaaggaacctcagtcaccgtctcctca

SEQ ID NO: 8 - protein, 107 aa, synthetic construct
  REGION 1..107: note = source = /note="Description of Artificial Sequence: Synthetic polypeptide"
DIVMTQSHKFMSTSVGDRVSITCKASQDVGTAVAWYQQKPGQSPKLLIYWASTRHTGVPDRFTGSGSGTDFTLTISNVQSEDLADYFCQQYNSYPLTFGAGSKLELK

SEQ ID NO: 9 - protein, 11 aa, synthetic construct
  REGION 1..11: note = source = /note="Description of Artificial Sequence: Synthetic peptide"
KASQDVGTAVA

SEQ ID NO: 10 - protein, 7 aa, synthetic construct
  REGION 1..7: note = source = /note="Description of Artificial Sequence: Synthetic peptide"
WASTRHT

SEQ ID NO: 11 - protein, 9 aa, synthetic construct
  REGION 1..9: note = source = /note="Description of Artificial Sequence: Synthetic peptide"
QQYNSYPLT

SEQ ID NO: 12 - protein, 7 aa, synthetic construct
  REGION 1..7: note = source = /note="Description of Artificial Sequence: Synthetic peptide"
SQDVGTA

SEQ ID NO: 13 - skipped

SEQ ID NO: 14 - protein, 6 aa, synthetic construct
  REGION 1..6: note = source = /note="Description of Artificial Sequence: Synthetic peptide"
YNSYPL

SEQ ID NO: 15 - DNA, 321 bp, synthetic construct
  misc_feature 1..321: note = source = /note="Description of Artificial Sequence: Synthetic polynucleotide"
  source 1..321: mol_type = other DNA
gacattgtgatgacccagtctcacaaattcatgtccacatcagtaggagacagggtcagcatcacctgcaaggccagtcaggatgtgggtactgctgtagcctggtatcaacagaaaccagggcaatctcctaaactactgatttactgggcatccacccggcacactggagtccctgatcgcttcacaggcagtggatctgggacagatttcactctcaccattagcaatgtgcagtctgaagacttggcagattatttctgtcagcagtataacagctatcctctcacgttcggtgctgggtccaagctggagctgaaa

SEQ ID NO: 16 - protein, 120 aa, synthetic construct
  REGION 1..120: note = source = /note="Description of Artificial Sequence: Synthetic polypeptide"
EVQLQQSGAELVKPGASVKLSCKASGYTFTSYWMYWVKQGPGRGLEWIGRIDPNSGSTKYNEKFKNKATLTVDKSSSTAYMQLSSLTSEDSAVYYCARDYRKGLYAMDYWGQGTTVTVSS

SEQ ID NO: 17 - protein, 107 aa, synthetic construct
  REGION 1..107: note = source = /note="Description of Artificial Sequence: Synthetic polypeptide"
DIMMTQSHKFMSTSVGDRVSITCKASQDVGTAVAWYQQKPGQSPKLLIYWASTRHTGVPDRFTGSGSGTDFTLTISNVQSEDLADYFCQQYNSYPLTFGQGTKVEIK

SEQ ID NO: 18 - protein, 120 aa, synthetic construct
  REGION 1..120: note = source = /note="Description of Artificial Sequence: Synthetic polypeptide"
QVQLVQSGAEVKKPGASVKVSCKASGYTFTSYWMYWVRQATGQGLEWMGRIDPNSGSTKYNEKFKNRFTISRDDSKNTAYLQMNSLKTEDTAVYYCARDYRKGLYAMDYWGQGTTVTVSS

SEQ ID NO: 19 - DNA, 360 bp, synthetic construct
  misc_feature 1..360: note = source = /note="Description of Artificial Sequence: Synthetic polynucleotide"
  source 1..360: mol_type = other DNA
caggttcagctggtgcagtctggagctgaggtgaagaagcctggggcctcagtgaaggtctcctgcaaggcttctggctacaccttcaccagttactggatgtactgggtgcgacaggccactggacaagggcttgagtggatgggtaggattgatcctaatagtgggagtactaagtacaatgagaagttcaagaacagattcaccatctccagagatgattcaaagaacacggcgtatctgcaaatgaacagcctgaaaaccgaggacacggccgtgtattactgtgcaagggactatagaaaggggctctatgctatggactactggggccagggcaccaccgtgaccgtgtcctcc

SEQ ID NO: 20 - protein, 447 aa, synthetic construct
  REGION 1..447: note = source = /note="Description of Artificial Sequence: Synthetic polypeptide"
QVQLVQSGAEVKKPGASVKVSCKASGYTFTSYWMYWVRQATGQGLEWMGRIDPNSGSTKYNEKFKNRFTISRDDSKNTAYLQMNSLKTEDTAVYYCARDYRKGLYAMDYWGQGTTVTVSSASTKGPSVFPLAPCSRSTSESTAALGCLVKDYFPEPVTVSWNSGALTSGVHTFPAVLQSSGLYSLSSVVTVPSSSLGTKTYTCNVDHKPSNTKVDKRVESKYGPPCPPCPAPEFLGGPSVFLFPPKPKDTLMISRTPEVTCVVVDVSQEDPEVQFNWYVDGVEVHNAKTKPREEQFNSTYRVVSVLTVLHQDWLNGKEYKCKVSNKGLPSSIEKTISKAKGQPREPQVYTLPPSQEEMTKNQVSLTCLVKGFYPSDIAVEWESNGQPENNYKTTPPVLDSDGSFFLYSRLTVDKSRWQEGNVFSCSVMHEALHNHYTQKSLSLSLGK

SEQ ID NO: 21 - DNA, 1341 bp, synthetic construct
  misc_feature 1..1341: note = source = /note="Description of Artificial Sequence: Synthetic polynucleotide"
  source 1..1341: mol_type = other DNA
caggttcagctggtgcagtctggagctgaggtgaagaagcctggggcctcagtgaaggtctcctgcaaggcttctggctacaccttcaccagttactggatgtactgggtgcgacaggccactggacaagggcttgagtggatgggtaggattgatcctaatagtgggagtactaagtacaatgagaagttcaagaacagattcaccatctccagagatgattcaaagaacacggcgtatctgcaaatgaacagcctgaaaaccgaggacacggccgtgtattactgtgcaagggactatagaaaggggctctatgctatggactactggggccagggcaccaccgtgaccgtgtcctccgcttccaccaagggcccatccgtcttccccctggcgccctgctccaggagcacctccgagagcacagccgccctgggctgcctggtcaaggactacttccccgaaccggtgacggtgtcgtggaactcaggcgccctgaccagcggcgtgcacaccttcccggctgtcctacagtcctcaggactctactccctcagcagcgtggtgaccgtgccctccagcagcttgggcacgaagacctacacctgcaacgtagatcacaagcccagcaacaccaaggtggacaagagagttgagtccaaatatggtcccccatgcccaccgtgcccagcacctgagttcctggggggaccatcagtcttcctgttccccccaaaacccaaggacactctcatgatctcccggacccctgaggtcacgtgcgtggtggtggacgtgagccaggaagaccccgaggtccagttcaactggtacgtggatggcgtggaggtgcataatgccaagacaaagccgcgggaggagcagttcaacagcacgtaccgtgtggtcagcgtcctcaccgtcctgcaccaggactggctgaacggcaaggagtacaagtgcaaggtgtccaacaaaggcctcccgtcctccatcgagaaaaccatctccaaagccaaagggcagccccgagagccacaggtgtacaccctgcccccatcccaggaggagatgaccaagaaccaggtcagcctgacctgcctggtcaaaggcttctaccccagcgacatcgccgtggagtgggagagcaatgggcagccggagaacaactacaagaccacgcctcccgtgctggactccgacggctccttcttcctctacagcaggctaaccgtggacaagagcaggtggcaggaggggaatgtcttctcatgctccgtgatgcatgaggctctgcacaaccactacacacagaagagcctctccctgtctctgggtaaa

SEQ ID NO: 22 - protein, 107 aa, synthetic construct
  REGION 1..107: note = source = /note="Description of Artificial Sequence: Synthetic polypeptide"
DIVMTQTPLSLPVTPGEPASISCKASQDVGTAVAWYLQKPGQSPQLLIYWASTRHTGIPARFSGSGSGTEFTLTISSLQSEDFAVYYCQQYNSYPLTFGQGTKVEIK

SEQ ID NO: 23 - DNA, 321 bp, synthetic construct
  misc_feature 1..321: note = source = /note="Description of Artificial Sequence: Synthetic polynucleotide"
  source 1..321: mol_type = other DNA
gatattgtgatgacccagactccactctccctgcccgtcacccctggagagccggcctccatctcctgcaaggccagtcaggatgtgggtactgctgtagcctggtacctgcagaagccagggcagtctccacagctcctgatctattgggcatccacccggcacactgggatcccagccaggttcagtggcagtgggtctgggacagagttcactctcaccatcagcagcctgcagtctgaagattttgcagtttattactgtcagcagtataacagctatcctctcacgttcggccaagggaccaaggtggaaatcaaa

SEQ ID NO: 24 - protein, 214 aa, synthetic construct
  REGION 1..214: note = source = /note="Description of Artificial Sequence: Synthetic polypeptide"
DIVMTQTPLSLPVTPGEPASISCKASQDVGTAVAWYLQKPGQSPQLLIYWASTRHTGIPARFSGSGSGTEFTLTISSLQSEDFAVYYCQQYNSYPLTFGQGTKVEIKRTVAAPSVFIFPPSDEQLKSGTASVVCLLNNFYPREAKVQWKVDNALQSGNSQESVTEQDSKDSTYSLSSTLTLSKADYEKHKVYACEVTHQGLSSPVTKSFNRGEC

SEQ ID NO: 25 - DNA, 642 bp, synthetic construct
  misc_feature 1..642: note = source = /note="Description of Artificial Sequence: Synthetic polynucleotide"
  source 1..642: mol_type = other DNA
gatattgtgatgacccagactccactctccctgcccgtcacccctggagagccggcctccatctcctgcaaggccagtcaggatgtgggtactgctgtagcctggtacctgcagaagccagggcagtctccacagctcctgatctattgggcatccacccggcacactgggatcccagccaggttcagtggcagtgggtctgggacagagttcactctcaccatcagcagcctgcagtctgaagattttgcagtttattactgtcagcagtataacagctatcctctcacgttcggccaagggaccaaggtggaaatcaaacgtacggtggctgcaccatctgtcttcatcttcccgccatctgatgagcagttgaaatctggaactgcctctgttgtgtgcctgctgaataacttctatcccagagaggccaaagtacagtggaaggtggataacgccctccaatcgggtaactcccaggagagtgtcacagagcaggacagcaaggacagcacctacagcctcagcagcaccctgacgctgagcaaagcagactacgagaaacacaaagtctacgcctgcgaagtcacccatcagggcctgagctcgcccgtcacaaagagcttcaacaggggagagtgt

SEQ ID NO: 26 - protein, 107 aa, synthetic construct
  REGION 1..107: note = source = /note="Description of Artificial Sequence: Synthetic polypeptide"
DIQMTQSPSSLSASVGDRVTITCKASQDVGTAVAWYLQKPGQSPQLLIYWASTRHTGVPSRFSGSGSGTDFTLTISSLQPEDFATYYCQQYNSYPLTFGQGTKVEIK

SEQ ID NO: 27 - DNA, 321 bp, synthetic construct
  misc_feature 1..321: note = source = /note="Description of Artificial Sequence: Synthetic polynucleotide"
  source 1..321: mol_type = other DNA
gacatccagatgacccagtctccatcctccctgtctgcatctgtaggagacagagtcaccatcacttgcaaggccagtcaggatgtgggtactgctgtagcctggtacctgcagaagccagggcagtctccacagctcctgatctattgggcatccacccggcacactggggtcccatcaaggttcagcggcagtggatctgggacagatttcactctcaccatcagcagcctgcagcctgaagattttgcaacttattactgtcagcagtataacagctatcctctcacgttcggccaagggaccaaggtggaaatcaaa

SEQ ID NO: 28 - protein, 214 aa, synthetic construct
  REGION 1..214: note = source = /note="Description of Artificial Sequence: Synthetic polypeptide"
DIQMTQSPSSLSASVGDRVTITCKASQDVGTAVAWYLQKPGQSPQLLIYWASTRHTGVPSRFSGSGSGTDFTLTISSLQPEDFATYYCQQYNSYPLTFGQGTKVEIKRTVAAPSVFIFPPSDEQLKSGTASVVCLLNNFYPREAKVQWKVDNALQSGNSQESVTEQDSKDSTYSLSSTLTLSKADYEKHKVYACEVTHQGLSSPVTKSFNRGEC

SEQ ID NO: 29 - DNA, 642 bp, synthetic construct
  misc_feature 1..642: note = source = /note="Description of Artificial Sequence: Synthetic polynucleotide"
  source 1..642: mol_type = other DNA
gacatccagatgacccagtctccatcctccctgtctgcatctgtaggagacagagtcaccatcacttgcaaggccagtcaggatgtgggtactgctgtagcctggtacctgcagaagccagggcagtctccacagctcctgatctattgggcatccacccggcacactggggtcccatcaaggttcagcggcagtggatctgggacagatttcactctcaccatcagcagcctgcagcctgaagattttgcaacttattactgtcagcagtataacagctatcctctcacgttcggccaagggaccaaggtggaaatcaaacgtacggtggctgcaccatctgtcttcatcttcccgccatctgatgagcagttgaaatctggaactgcctctgttgtgtgcctgctgaataacttctatcccagagaggccaaagtacagtggaaggtggataacgccctccaatcgggtaactcccaggagagtgtcacagagcaggacagcaaggacagcacctacagcctcagcagcaccctgacgctgagcaaagcagactacgagaaacacaaagtctacgcctgcgaagtcacccatcagggcctgagctcgcccgtcacaaagagcttcaacaggggagagtgt

SEQ ID NO: 30 - protein, 120 aa, synthetic construct
  REGION 1..120: note = source = /note="Description of Artificial Sequence: Synthetic polypeptide"
EVQLVQSGAEVKKPGATVKISCKVSGYTFTSYWMYWVRQATGQGLEWMGRIDPNSGSTKYNEKFKNRVTITADKSTSTAYMELSSLRSEDTAVYYCARDYRKGLYAMDYWGQGTTVTVSS

SEQ ID NO: 31 - DNA, 360 bp, synthetic construct
  misc_feature 1..360: note = source = /note="Description of Artificial Sequence: Synthetic polynucleotide"
  source 1..360: mol_type = other DNA
gaggtccagctggtacagtctggggctgaggtgaagaagcctggggctacagtgaaaatctcctgcaaggtttctggctacaccttcaccagttactggatgtactgggtgcgacaggccactggacaagggcttgagtggatgggtaggattgatcctaatagtgggagtactaagtacaatgagaagttcaagaacagagtcacgattaccgcggacaaatccacgagcacagcctacatggagctgagcagcctgagatctgaggacacggccgtgtattactgtgcaagggactatagaaaggggctctatgctatggactactggggccagggcaccaccgtgaccgtgtcctcc

SEQ ID NO: 32 - protein, 447 aa, synthetic construct
  REGION 1..447: note = source = /note="Description of Artificial Sequence: Synthetic polypeptide"
EVQLVQSGAEVKKPGATVKISCKVSGYTFTSYWMYWVRQATGQGLEWMGRIDPNSGSTKYNEKFKNRVTITADKSTSTAYMELSSLRSEDTAVYYCARDYRKGLYAMDYWGQGTTVTVSSASTKGPSVFPLAPCSRSTSESTAALGCLVKDYFPEPVTVSWNSGALTSGVHTFPAVLQSSGLYSLSSVVTVPSSSLGTKTYTCNVDHKPSNTKVDKRVESKYGPPCPPCPAPEFLGGPSVFLFPPKPKDTLMISRTPEVTCVVVDVSQEDPEVQFNWYVDGVEVHNAKTKPREEQFNSTYRVVSVLTVLHQDWLNGKEYKCKVSNKGLPSSIEKTISKAKGQPREPQVYTLPPSQEEMTKNQVSLTCLVKGFYPSDIAVEWESNGQPENNYKTTPPVLDSDGSFFLYSRLTVDKSRWQEGNVFSCSVMHEALHNHYTQKSLSLSLGK

SEQ ID NO: 33 - DNA, 1341 bp, synthetic construct
  misc_feature 1..1341: note = source = /note="Description of Artificial Sequence: Synthetic polynucleotide"
  source 1..1341: mol_type = other DNA
gaggtccagctggtacagtctggggctgaggtgaagaagcctggggctacagtgaaaatctcctgcaaggtttctggctacaccttcaccagttactggatgtactgggtgcgacaggccactggacaagggcttgagtggatgggtaggattgatcctaatagtgggagtactaagtacaatgagaagttcaagaacagagtcacgattaccgcggacaaatccacgagcacagcctacatggagctgagcagcctgagatctgaggacacggccgtgtattactgtgcaagggactatagaaaggggctctatgctatggactactggggccagggcaccaccgtgaccgtgtcctccgcttccaccaagggcccatccgtcttccccctggcgccctgctccaggagcacctccgagagcacagccgccctgggctgcctggtcaaggactacttccccgaaccggtgacggtgtcgtggaactcaggcgccctgaccagcggcgtgcacaccttcccggctgtcctacagtcctcaggactctactccctcagcagcgtggtgaccgtgccctccagcagcttgggcacgaagacctacacctgcaacgtagatcacaagcccagcaacaccaaggtggacaagagagttgagtccaaatatggtcccccatgcccaccgtgcccagcacctgagttcctggggggaccatcagtcttcctgttccccccaaaacccaaggacactctcatgatctcccggacccctgaggtcacgtgcgtggtggtggacgtgagccaggaagaccccgaggtccagttcaactggtacgtggatggcgtggaggtgcataatgccaagacaaagccgcgggaggagcagttcaacagcacgtaccgtgtggtcagcgtcctcaccgtcctgcaccaggactggctgaacggcaaggagtacaagtgcaaggtgtccaacaaaggcctcccgtcctccatcgagaaaaccatctccaaagccaaagggcagccccgagagccacaggtgtacaccctgcccccatcccaggaggagatgaccaagaaccaggtcagcctgacctgcctggtcaaaggcttctaccccagcgacatcgccgtggagtgggagagcaatgggcagccggagaacaactacaagaccacgcctcccgtgctggactccgacggctccttcttcctctacagcaggctaaccgtggacaagagcaggtggcaggaggggaatgtcttctcatgctccgtgatgcatgaggctctgcacaaccactacacacagaagagcctctccctgtctctgggtaaa

SEQ ID NO: 34 - protein, 107 aa, synthetic construct
  REGION 1..107: note = source = /note="Description of Artificial Sequence: Synthetic polypeptide"
EIVLTQSPDFQSVTPKEKVTITCKASQDVGTAVAWYLQKPGQSPQLLIYWASTRHTGVPDRFSGSGSGTDFTLKISRVEAEDVGVYYCQQYNSYPLTFGQGTKVEIK

SEQ ID NO: 35 - DNA, 321 bp, synthetic construct
  misc_feature 1..321: note = source = /note="Description of Artificial Sequence: Synthetic polynucleotide"
  source 1..321: mol_type = other DNA
gaaattgtgctgactcagtctccagactttcagtctgtgactccaaaggagaaagtcaccatcacctgcaaggccagtcaggatgtgggtactgctgtagcctggtacctgcagaagccagggcagtctccacagctcctgatctattgggcatccacccggcacactggggtcccagacaggttcagtggcagtgggtcaggcactgatttcacactgaaaatcagcagggtggaggctgaggatgttggagtttattactgtcagcagtataacagctatcctctcacgttcggccaagggaccaaggtggaaatcaaa

SEQ ID NO: 36 - protein, 214 aa, synthetic construct
  REGION 1..214: note = source = /note="Description of Artificial Sequence: Synthetic polypeptide"
EIVLTQSPDFQSVTPKEKVTITCKASQDVGTAVAWYLQKPGQSPQLLIYWASTRHTGVPDRFSGSGSGTDFTLKISRVEAEDVGVYYCQQYNSYPLTFGQGTKVEIKRTVAAPSVFIFPPSDEQLKSGTASVVCLLNNFYPREAKVQWKVDNALQSGNSQESVTEQDSKDSTYSLSSTLTLSKADYEKHKVYACEVTHQGLSSPVTKSFNRGEC

SEQ ID NO: 37 - DNA, 642 bp, synthetic construct
  misc_feature 1..642: note = source = /note="Description of Artificial Sequence: Synthetic polynucleotide"
  source 1..642: mol_type = other DNA
gaaattgtgctgactcagtctccagactttcagtctgtgactccaaaggagaaagtcaccatcacctgcaaggccagtcaggatgtgggtactgctgtagcctggtacctgcagaagccagggcagtctccacagctcctgatctattgggcatccacccggcacactggggtcccagacaggttcagtggcagtgggtcaggcactgatttcacactgaaaatcagcagggtggaggctgaggatgttggagtttattactgtcagcagtataacagctatcctctcacgttcggccaagggaccaaggtggaaatcaaacgtacggtggctgcaccatctgtcttcatcttcccgccatctgatgagcagttgaaatctggaactgcctctgttgtgtgcctgctgaataacttctatcccagagaggccaaagtacagtggaaggtggataacgccctccaatcgggtaactcccaggagagtgtcacagagcaggacagcaaggacagcacctacagcctcagcagcaccctgacgctgagcaaagcagactacgagaaacacaaagtctacgcctgcgaagtcacccatcagggcctgagctcgcccgtcacaaagagcttcaacaggggagagtgt

SEQ ID NO: 38 - protein, 120 aa, synthetic construct
  REGION 1..120: note = source = /note="Description of Artificial Sequence: Synthetic polypeptide"
EVQLVQSGAEVKKPGESLRISCKGSGYTFTSYWMYWVRQAPGQGLEWMGRIDPNSGSTKYNEKFKNRVTISVDTSKNQFSLKLSSVTAADTAVYYCARDYRKGLYAMDYWGQGTTVTVSS

SEQ ID NO: 39 - DNA, 360 bp, synthetic construct
  misc_feature 1..360: note = source = /note="Description of Artificial Sequence: Synthetic polynucleotide"
  source 1..360: mol_type = other DNA
gaagtgcagctggtgcagtctggagcagaggtgaaaaagcccggggagtctctgaggatctcctgtaagggttctggctacaccttcaccagttactggatgtactgggtgcgacaggcccctggacaagggcttgagtggatgggtaggattgatcctaatagtgggagtactaagtacaatgagaagttcaagaacagagtcaccatatcagtagacacgtccaagaaccagttctccctgaagctgagctctgtgaccgccgcggacacggctgtgtattactgtgcaagggactatagaaaggggctctatgctatggactactggggccagggcaccaccgtgaccgtgtcctcc

SEQ ID NO: 40 - protein, 447 aa, synthetic construct
  REGION 1..447: note = source = /note="Description of Artificial Sequence: Synthetic polypeptide"
EVQLVQSGAEVKKPGESLRISCKGSGYTFTSYWMYWVRQAPGQGLEWMGRIDPNSGSTKYNEKFKNRVTISVDTSKNQFSLKLSSVTAADTAVYYCARDYRKGLYAMDYWGQGTTVTVSSASTKGPSVFPLAPCSRSTSESTAALGCLVKDYFPEPVTVSWNSGALTSGVHTFPAVLQSSGLYSLSSVVTVPSSSLGTKTYTCNVDHKPSNTKVDKRVESKYGPPCPPCPAPEFLGGPSVFLFPPKPKDTLMISRTPEVTCVVVDVSQEDPEVQFNWYVDGVEVHNAKTKPREEQFNSTYRVVSVLTVLHQDWLNGKEYKCKVSNKGLPSSIEKTISKAKGQPREPQVYTLPPSQEEMTKNQVSLTCLVKGFYPSDIAVEWESNGQPENNYKTTPPVLDSDGSFFLYSRLTVDKSRWQEGNVFSCSVMHEALHNHYTQKSLSLSLGK

SEQ ID NO: 41 - DNA, 1341 bp, synthetic construct
  misc_feature 1..1341: note = source = /note="Description of Artificial Sequence: Synthetic polynucleotide"
  source 1..1341: mol_type = other DNA
gaagtgcagctggtgcagtctggagcagaggtgaaaaagcccggggagtctctgaggatctcctgtaagggttctggctacaccttcaccagttactggatgtactgggtgcgacaggcccctggacaagggcttgagtggatgggtaggattgatcctaatagtgggagtactaagtacaatgagaagttcaagaacagagtcaccatatcagtagacacgtccaagaaccagttctccctgaagctgagctctgtgaccgccgcggacacggctgtgtattactgtgcaagggactatagaaaggggctctatgctatggactactggggccagggcaccaccgtgaccgtgtcctccgcttccaccaagggcccatccgtcttccccctggcgccctgctccaggagcacctccgagagcacagccgccctgggctgcctggtcaaggactacttccccgaaccggtgacggtgtcgtggaactcaggcgccctgaccagcggcgtgcacaccttcccggctgtcctacagtcctcaggactctactccctcagcagcgtggtgaccgtgccctccagcagcttgggcacgaagacctacacctgcaacgtagatcacaagcccagcaacaccaaggtggacaagagagttgagtccaaatatggtcccccatgcccaccgtgcccagcacctgagttcctggggggaccatcagtcttcctgttccccccaaaacccaaggacactctcatgatctcccggacccctgaggtcacgtgcgtggtggtggacgtgagccaggaagaccccgaggtccagttcaactggtacgtggatggcgtggaggtgcataatgccaagacaaagccgcgggaggagcagttcaacagcacgtaccgtgtggtcagcgtcctcaccgtcctgcaccaggactggctgaacggcaaggagtacaagtgcaaggtgtccaacaaaggcctcccgtcctccatcgagaaaaccatctccaaagccaaagggcagccccgagagccacaggtgtacaccctgcccccatcccaggaggagatgaccaagaaccaggtcagcctgacctgcctggtcaaaggcttctaccccagcgacatcgccgtggagtgggagagcaatgggcagccggagaacaactacaagaccacgcctcccgtgctggactccgacggctccttcttcctctacagcaggctaaccgtggacaagagcaggtggcaggaggggaatgtcttctcatgctccgtgatgcatgaggctctgcacaaccactacacacagaagagcctctccctgtctctgggtaaa

SEQ ID NO: 42 - protein, 107 aa, synthetic construct
  REGION 1..107: note = source = /note="Description of Artificial Sequence: Synthetic polypeptide"
EIVLTQSPDFQSVTPKEKVTITCKASQDVGTAVAWYLQKPGQSPQLLIYWASTRHTGVPSRFSGSGSGTDFTFTISSLQPEDIATYYCQQYNSYPLTFGQGTKVEIK

SEQ ID NO: 43 - DNA, 321 bp, synthetic construct
  misc_feature 1..321: note = source = /note="Description of Artificial Sequence: Synthetic polynucleotide"
  source 1..321: mol_type = other DNA
gaaattgtgctgactcagtctccagactttcagtctgtgactccaaaggagaaagtcaccatcacctgcaaggccagtcaggatgtgggtactgctgtagcctggtacctgcagaagccagggcagtctccacagctcctgatctattgggcatccacccggcacactggggtcccatcaaggttcagtggaagtggatctgggacagattttactttcaccatcagcagcctgcagcctgaagatattgcaacatattactgtcagcagtataacagctatcctctcacgttcggccaagggaccaaggtggaaatcaaa

SEQ ID NO: 44 - protein, 214 aa, synthetic construct
  REGION 1..214: note = source = /note="Description of Artificial Sequence: Synthetic polypeptide"
EIVLTQSPDFQSVTPKEKVTITCKASQDVGTAVAWYLQKPGQSPQLLIYWASTRHTGVPSRFSGSGSGTDFTFTISSLQPEDIATYYCQQYNSYPLTFGQGTKVEIKRTVAAPSVFIFPPSDEQLKSGTASVVCLLNNFYPREAKVQWKVDNALQSGNSQESVTEQDSKDSTYSLSSTLTLSKADYEKHKVYACEVTHQGLSSPVTKSFNRGEC

SEQ ID NO: 45 - DNA, 642 bp, synthetic construct
  misc_feature 1..642: note = source = /note="Description of Artificial Sequence: Synthetic polynucleotide"
  source 1..642: mol_type = other DNA
gaaattgtgctgactcagtctccagactttcagtctgtgactccaaaggagaaagtcaccatcacctgcaaggccagtcaggatgtgggtactgctgtagcctggtacctgcagaagccagggcagtctccacagctcctgatctattgggcatccacccggcacactggggtcccatcaaggttcagtggaagtggatctgggacagattttactttcaccatcagcagcctgcagcctgaagatattgcaacatattactgtcagcagtataacagctatcctctcacgttcggccaagggaccaaggtggaaatcaaacgtacggtggctgcaccatctgtcttcatcttcccgccatctgatgagcagttgaaatctggaactgcctctgttgtgtgcctgctgaataacttctatcccagagaggccaaagtacagtggaaggtggataacgccctccaatcgggtaactcccaggagagtgtcacagagcaggacagcaaggacagcacctacagcctcagcagcaccctgacgctgagcaaagcagactacgagaaacacaaagtctacgcctgcgaagtcacccatcagggcctgagctcgcccgtcacaaagagcttcaacaggggagagtgt

SEQ ID NO: 46 - protein, 120 aa, synthetic construct
  REGION 1..120: note = source = /note="Description of Artificial Sequence: Synthetic polypeptide"
EVQLVQSGAEVKKPGATVKISCKVSGYTFTSYWMYWIRQSPSRGLEWLGRIDPNSGSTKYNEKFKNRLTISKDTSKNQVVLTMTNMDPVDTATYYCARDYRKGLYAMDYWGQGTTVTVSS

SEQ ID NO: 47 - DNA, 360 bp, synthetic construct
  misc_feature 1..360: note = source = /note="Description of Artificial Sequence: Synthetic polynucleotide"
  source 1..360: mol_type = other DNA
gaggtccagctggtacagtctggggctgaggtgaagaagcctggggctacagtgaaaatctcctgcaaggtttctggctacaccttcaccagttactggatgtactggatcaggcagtccccatcgagaggccttgagtggctgggtaggattgatcctaatagtgggagtactaagtacaatgagaagttcaagaacagactcaccatctccaaggacacctccaaaaaccaggtggtccttacaatgaccaacatggaccctgtggacacagccacgtattactgtgcaagggactatagaaaggggctctatgctatggactactggggccagggcaccaccgtgaccgtgtcctcc

SEQ ID NO: 48 - protein, 447 aa, synthetic construct
  REGION 1..447: note = source = /note="Description of Artificial Sequence: Synthetic polypeptide"
EVQLVQSGAEVKKPGATVKISCKVSGYTFTSYWMYWIRQSPSRGLEWLGRIDPNSGSTKYNEKFKNRLTISKDTSKNQVVLTMTNMDPVDTATYYCARDYRKGLYAMDYWGQGTTVTVSSASTKGPSVFPLAPCSRSTSESTAALGCLVKDYFPEPVTVSWNSGALTSGVHTFPAVLQSSGLYSLSSVVTVPSSSLGTKTYTCNVDHKPSNTKVDKRVESKYGPPCPPCPAPEFLGGPSVFLFPPKPKDTLMISRTPEVTCVVVDVSQEDPEVQFNWYVDGVEVHNAKTKPREEQFNSTYRVVSVLTVLHQDWLNGKEYKCKVSNKGLPSSIEKTISKAKGQPREPQVYTLPPSQEEMTKNQVSLTCLVKGFYPSDIAVEWESNGQPENNYKTTPPVLDSDGSFFLYSRLTVDKSRWQEGNVFSCSVMHEALHNHYTQKSLSLSLGK

SEQ ID NO: 49 - DNA, 1341 bp, synthetic construct
  misc_feature 1..1341: note = source = /note="Description of Artificial Sequence: Synthetic polynucleotide"
  source 1..1341: mol_type = other DNA
gaggtccagctggtacagtctggggctgaggtgaagaagcctggggctacagtgaaaatctcctgcaaggtttctggctacaccttcaccagttactggatgtactggatcaggcagtccccatcgagaggccttgagtggctgggtaggattgatcctaatagtgggagtactaagtacaatgagaagttcaagaacagactcaccatctccaaggacacctccaaaaaccaggtggtccttacaatgaccaacatggaccctgtggacacagccacgtattactgtgcaagggactatagaaaggggctctatgctatggactactggggccagggcaccaccgtgaccgtgtcctccgcttccaccaagggcccatccgtcttccccctggcgccctgctccaggagcacctccgagagcacagccgccctgggctgcctggtcaaggactacttccccgaaccggtgacggtgtcgtggaactcaggcgccctgaccagcggcgtgcacaccttcccggctgtcctacagtcctcaggactctactccctcagcagcgtggtgaccgtgccctccagcagcttgggcacgaagacctacacctgcaacgtagatcacaagcccagcaacaccaaggtggacaagagagttgagtccaaatatggtcccccatgcccaccgtgcccagcacctgagttcctggggggaccatcagtcttcctgttccccccaaaacccaaggacactctcatgatctcccggacccctgaggtcacgtgcgtggtggtggacgtgagccaggaagaccccgaggtccagttcaactggtacgtggatggcgtggaggtgcataatgccaagacaaagccgcgggaggagcagttcaacagcacgtaccgtgtggtcagcgtcctcaccgtcctgcaccaggactggctgaacggcaaggagtacaagtgcaaggtgtccaacaaaggcctcccgtcctccatcgagaaaaccatctccaaagccaaagggcagccccgagagccacaggtgtacaccctgcccccatcccaggaggagatgaccaagaaccaggtcagcctgacctgcctggtcaaaggcttctaccccagcgacatcgccgtggagtgggagagcaatgggcagccggagaacaactacaagaccacgcctcccgtgctggactccgacggctccttcttcctctacagcaggctaaccgtggacaagagcaggtggcaggaggggaatgtcttctcatgctccgtgatgcatgaggctctgcacaaccactacacacagaagagcctctccctgtctctgggtaaa

SEQ ID NO: 50 - protein, 120 aa, synthetic construct
  REGION 1..120: note = source = /note="Description of Artificial Sequence: Synthetic polypeptide"
EVQLVQSGAEVKKPGESLRISCKGSGYTFTSYWMYWIRQPPGKGLEWIGRIDPNSGSTKYNEKFKNRVTITADKSTSTAYMELSSLRSEDTAVYYCARDYRKGLYAMDYWGQGTTVTVSS

SEQ ID NO: 51 - DNA, 360 bp, synthetic construct
  misc_feature 1..360: note = source = /note="Description of Artificial Sequence: Synthetic polynucleotide"
  source 1..360: mol_type = other DNA
gaagtgcagctggtgcagtctggagcagaggtgaaaaagcccggggagtctctgaggatctcctgtaagggttctggctacaccttcaccagttactggatgtactggatccgccagcccccagggaaggggctggagtggattggtaggattgatcctaatagtgggagtactaagtacaatgagaagttcaagaacagagtcacgattaccgcggacaaatccacgagcacagcctacatggagctgagcagcctgagatctgaggacacggccgtgtattactgtgcaagggactatagaaaggggctctatgctatggactactggggccagggcaccaccgtgaccgtgtcctcc

SEQ ID NO: 52 - protein, 447 aa, synthetic construct
  REGION 1..447: note = source = /note="Description of Artificial Sequence: Synthetic polypeptide"
EVQLVQSGAEVKKPGESLRISCKGSGYTFTSYWMYWIRQPPGKGLEWIGRIDPNSGSTKYNEKFKNRVTITADKSTSTAYMELSSLRSEDTAVYYCARDYRKGLYAMDYWGQGTTVTVSSASTKGPSVFPLAPCSRSTSESTAALGCLVKDYFPEPVTVSWNSGALTSGVHTFPAVLQSSGLYSLSSVVTVPSSSLGTKTYTCNVDHKPSNTKVDKRVESKYGPPCPPCPAPEFLGGPSVFLFPPKPKDTLMISRTPEVTCVVVDVSQEDPEVQFNWYVDGVEVHNAKTKPREEQFNSTYRVVSVLTVLHQDWLNGKEYKCKVSNKGLPSSIEKTISKAKGQPREPQVYTLPPSQEEMTKNQVSLTCLVKGFYPSDIAVEWESNGQPENNYKTTPPVLDSDGSFFLYSRLTVDKSRWQEGNVFSCSVMHEALHNHYTQKSLSLSLGK

SEQ ID NO: 53 - DNA, 1341 bp, synthetic construct
  misc_feature 1..1341: note = source = /note="Description of Artificial Sequence: Synthetic polynucleotide"
  source 1..1341: mol_type = other DNA
gaagtgcagctggtgcagtctggagcagaggtgaaaaagcccggggagtctctgaggatctcctgtaagggttctggctacaccttcaccagttactggatgtactggatccgccagcccccagggaaggggctggagtggattggtaggattgatcctaatagtgggagtactaagtacaatgagaagttcaagaacagagtcacgattaccgcggacaaatccacgagcacagcctacatggagctgagcagcctgagatctgaggacacggccgtgtattactgtgcaagggactatagaaaggggctctatgctatggactactggggccagggcaccaccgtgaccgtgtcctccgcttccaccaagggcccatccgtcttccccctggcgccctgctccaggagcacctccgagagcacagccgccctgggctgcctggtcaaggactacttccccgaaccggtgacggtgtcgtggaactcaggcgccctgaccagcggcgtgcacaccttcccggctgtcctacagtcctcaggactctactccctcagcagcgtggtgaccgtgccctccagcagcttgggcacgaagacctacacctgcaacgtagatcacaagcccagcaacaccaaggtggacaagagagttgagtccaaatatggtcccccatgcccaccgtgcccagcacctgagttcctggggggaccatcagtcttcctgttccccccaaaacccaaggacactctcatgatctcccggacccctgaggtcacgtgcgtggtggtggacgtgagccaggaagaccccgaggtccagttcaactggtacgtggatggcgtggaggtgcataatgccaagacaaagccgcgggaggagcagttcaacagcacgtaccgtgtggtcagcgtcctcaccgtcctgcaccaggactggctgaacggcaaggagtacaagtgcaaggtgtccaacaaaggcctcccgtcctccatcgagaaaaccatctccaaagccaaagggcagccccgagagccacaggtgtacaccctgcccccatcccaggaggagatgaccaagaaccaggtcagcctgacctgcctggtcaaaggcttctaccccagcgacatcgccgtggagtgggagagcaatgggcagccggagaacaactacaagaccacgcctcccgtgctggactccgacggctccttcttcctctacagcaggctaaccgtggacaagagcaggtggcaggaggggaatgtcttctcatgctccgtgatgcatgaggctctgcacaaccactacacacagaagagcctctccctgtctctgggtaaa

SEQ ID NO: 54 - protein, 120 aa, synthetic construct
  REGION 1..120: note = source = /note="Description of Artificial Sequence: Synthetic polypeptide"
QVQLVQSGAEVKKPGASVKVSCKASGYTFTSYWMYWIRQSPSRGLEWLGRIDPNSGSTKYNEKFKNRFTISRDDSKNTAYLQMNSLKTEDTAVYYCARDYRKGLYAMDYWGQGTTVTVSS

SEQ ID NO: 55 - DNA, 360 bp, synthetic construct
  misc_feature 1..360: note = source = /note="Description of Artificial Sequence: Synthetic polynucleotide"
  source 1..360: mol_type = other DNA
caggttcagctggtgcagtctggagctgaggtgaagaagcctggggcctcagtgaaggtctcctgcaaggcttctggctacaccttcaccagttactggatgtactggatcaggcagtccccatcgagaggccttgagtggctgggtaggattgatcctaatagtgggagtactaagtacaatgagaagttcaagaacagattcaccatctccagagatgattcaaagaacacggcgtatctgcaaatgaacagcctgaaaaccgaggacacggccgtgtattactgtgcaagggactatagaaaggggctctatgctatggactactggggccagggcaccaccgtgaccgtgtcctcc

SEQ ID NO: 56 - protein, 447 aa, synthetic construct
  REGION 1..447: note = source = /note="Description of Artificial Sequence: Synthetic polypeptide"
QVQLVQSGAEVKKPGASVKVSCKASGYTFTSYWMYWIRQSPSRGLEWLGRIDPNSGSTKYNEKFKNRFTISRDDSKNTAYLQMNSLKTEDTAVYYCARDYRKGLYAMDYWGQGTTVTVSSASTKGPSVFPLAPCSRSTSESTAALGCLVKDYFPEPVTVSWNSGALTSGVHTFPAVLQSSGLYSLSSVVTVPSSSLGTKTYTCNVDHKPSNTKVDKRVESKYGPPCPPCPAPEFLGGPSVFLFPPKPKDTLMISRTPEVTCVVVDVSQEDPEVQFNWYVDGVEVHNAKTKPREEQFNSTYRVVSVLTVLHQDWLNGKEYKCKVSNKGLPSSIEKTISKAKGQPREPQVYTLPPSQEEMTKNQVSLTCLVKGFYPSDIAVEWESNGQPENNYKTTPPVLDSDGSFFLYSRLTVDKSRWQEGNVFSCSVMHEALHNHYTQKSLSLSLGK

SEQ ID NO: 57 - DNA, 1341 bp, synthetic construct
  misc_feature 1..1341: note = source = /note="Description of Artificial Sequence: Synthetic polynucleotide"
  source 1..1341: mol_type = other DNA
caggttcagctggtgcagtctggagctgaggtgaagaagcctggggcctcagtgaaggtctcctgcaaggcttctggctacaccttcaccagttactggatgtactggatcaggcagtccccatcgagaggccttgagtggctgggtaggattgatcctaatagtgggagtactaagtacaatgagaagttcaagaacagattcaccatctccagagatgattcaaagaacacggcgtatctgcaaatgaacagcctgaaaaccgaggacacggccgtgtattactgtgcaagggactatagaaaggggctctatgctatggactactggggccagggcaccaccgtgaccgtgtcctccgcttccaccaagggcccatccgtcttccccctggcgccctgctccaggagcacctccgagagcacagccgccctgggctgcctggtcaaggactacttccccgaaccggtgacggtgtcgtggaactcaggcgccctgaccagcggcgtgcacaccttcccggctgtcctacagtcctcaggactctactccctcagcagcgtggtgaccgtgccctccagcagcttgggcacgaagacctacacctgcaacgtagatcacaagcccagcaacaccaaggtggacaagagagttgagtccaaatatggtcccccatgcccaccgtgcccagcacctgagttcctggggggaccatcagtcttcctgttccccccaaaacccaaggacactctcatgatctcccggacccctgaggtcacgtgcgtggtggtggacgtgagccaggaagaccccgaggtccagttcaactggtacgtggatggcgtggaggtgcataatgccaagacaaagccgcgggaggagcagttcaacagcacgtaccgtgtggtcagcgtcctcaccgtcctgcaccaggactggctgaacggcaaggagtacaagtgcaaggtgtccaacaaaggcctcccgtcctccatcgagaaaaccatctccaaagccaaagggcagccccgagagccacaggtgtacaccctgcccccatcccaggaggagatgaccaagaaccaggtcagcctgacctgcctggtcaaaggcttctaccccagcgacatcgccgtggagtgggagagcaatgggcagccggagaacaactacaagaccacgcctcccgtgctggactccgacggctccttcttcctctacagcaggctaaccgtggacaagagcaggtggcaggaggggaatgtcttctcatgctccgtgatgcatgaggctctgcacaaccactacacacagaagagcctctccctgtctctgggtaaa

SEQ ID NO: 58 - protein, 107 aa, synthetic construct
  REGION 1..107: note = source = /note="Description of Artificial Sequence: Synthetic polypeptide"
EIVLTQSPATLSLSPGERATLSCKASQDVGTAVAWYLQKPGQSPQLLIYWASTRHTGIPPRFSGSGYGTDFTLTINNIESEDAAYYFCQQYNSYPLTFGQGTKVEIK

SEQ ID NO: 59 - DNA, 321 bp, synthetic construct
  misc_feature 1..321: note = source = /note="Description of Artificial Sequence: Synthetic polynucleotide"
  source 1..321: mol_type = other DNA
gaaattgtgttgacacagtctccagccaccctgtctttgtctccaggggaaagagccaccctctcctgcaaggccagtcaggatgtgggtactgctgtagcctggtacctgcagaagccagggcagtctccacagctcctgatctattgggcatccacccggcacactgggatcccacctcgattcagtggcagcgggtatggaacagattttaccctcacaattaataacatagaatctgaggatgctgcatattacttctgtcagcagtataacagctatcctctcacgttcggccaagggaccaaggtggaaatcaaa

SEQ ID NO: 60 - protein, 214 aa, synthetic construct
  REGION 1..214: note = source = /note="Description of Artificial Sequence: Synthetic polypeptide"
EIVLTQSPATLSLSPGERATLSCKASQDVGTAVAWYLQKPGQSPQLLIYWASTRHTGIPPRFSGSGYGTDFTLTINNIESEDAAYYFCQQYNSYPLTFGQGTKVEIKRTVAAPSVFIFPPSDEQLKSGTASVVCLLNNFYPREAKVQWKVDNALQSGNSQESVTEQDSKDSTYSLSSTLTLSKADYEKHKVYACEVTHQGLSSPVTKSFNRGEC

SEQ ID NO: 61 - DNA, 642 bp, synthetic construct
  misc_feature 1..642: note = source = /note="Description of Artificial Sequence: Synthetic polynucleotide"
  source 1..642: mol_type = other DNA
gaaattgtgttgacacagtctccagccaccctgtctttgtctccaggggaaagagccaccctctcctgcaaggccagtcaggatgtgggtactgctgtagcctggtacctgcagaagccagggcagtctccacagctcctgatctattgggcatccacccggcacactgggatcccacctcgattcagtggcagcgggtatggaacagattttaccctcacaattaataacatagaatctgaggatgctgcatattacttctgtcagcagtataacagctatcctctcacgttcggccaagggaccaaggtggaaatcaaacgtacggtggctgcaccatctgtcttcatcttcccgccatctgatgagcagttgaaatctggaactgcctctgttgtgtgcctgctgaataacttctatcccagagaggccaaagtacagtggaaggtggataacgccctccaatcgggtaactcccaggagagtgtcacagagcaggacagcaaggacagcacctacagcctcagcagcaccctgacgctgagcaaagcagactacgagaaacacaaagtctacgcctgcgaagtcacccatcagggcctgagctcgcccgtcacaaagagcttcaacaggggagagtgt

SEQ ID NO: 62 - protein, 120 aa, synthetic construct
  REGION 1..120: note = source = /note="Description of Artificial Sequence: Synthetic polypeptide"
EVQLVQSGAEVKKPGESLRISCKGSGYTFTSYWMYWVRQARGQRLEWIGRIDPNSGSTKYNEKFKNRLTISKDTSKNQVVLTMTNMDPVDTATYYCARDYRKGLYAMDYWGQGTTVTVSS

SEQ ID NO: 63 - DNA, 360 bp, synthetic construct
  misc_feature 1..360: note = source = /note="Description of Artificial Sequence: Synthetic polynucleotide"
  source 1..360: mol_type = other DNA
gaagtgcagctggtgcagtctggagcagaggtgaaaaagcccggggagtctctgaggatctcctgtaagggttctggctacaccttcaccagttactggatgtactgggtgcgacaggctcgtggacaacgccttgagtggataggtaggattgatcctaatagtgggagtactaagtacaatgagaagttcaagaacagactcaccatctccaaggacacctccaaaaaccaggtggtccttacaatgaccaacatggaccctgtggacacagccacgtattactgtgcaagggactatagaaaggggctctatgctatggactactggggccagggcaccaccgtgaccgtgtcctcc

SEQ ID NO: 64 - protein, 447 aa, synthetic construct
  REGION 1..447: note = source = /note="Description of Artificial Sequence: Synthetic polypeptide"
EVQLVQSGAEVKKPGESLRISCKGSGYTFTSYWMYWVRQARGQRLEWIGRIDPNSGSTKYNEKFKNRLTISKDTSKNQVVLTMTNMDPVDTATYYCARDYRKGLYAMDYWGQGTTVTVSSASTKGPSVFPLAPCSRSTSESTAALGCLVKDYFPEPVTVSWNSGALTSGVHTFPAVLQSSGLYSLSSVVTVPSSSLGTKTYTCNVDHKPSNTKVDKRVESKYGPPCPPCPAPEFLGGPSVFLFPPKPKDTLMISRTPEVTCVVVDVSQEDPEVQFNWYVDGVEVHNAKTKPREEQFNSTYRVVSVLTVLHQDWLNGKEYKCKVSNKGLPSSIEKTISKAKGQPREPQVYTLPPSQEEMTKNQVSLTCLVKGFYPSDIAVEWESNGQPENNYKTTPPVLDSDGSFFLYSRLTVDKSRWQEGNVFSCSVMHEALHNHYTQKSLSLSLGK

SEQ ID NO: 65 - DNA, 1341 bp, synthetic construct
  misc_feature 1..1341: note = source = /note="Description of Artificial Sequence: Synthetic polynucleotide"
  source 1..1341: mol_type = other DNA
gaagtgcagctggtgcagtctggagcagaggtgaaaaagcccggggagtctctgaggatctcctgtaagggttctggctacaccttcaccagttactggatgtactgggtgcgacaggctcgtggacaacgccttgagtggataggtaggattgatcctaatagtgggagtactaagtacaatgagaagttcaagaacagactcaccatctccaaggacacctccaaaaaccaggtggtccttacaatgaccaacatggaccctgtggacacagccacgtattactgtgcaagggactatagaaaggggctctatgctatggactactggggccagggcaccaccgtgaccgtgtcctccgcttccaccaagggcccatccgtcttccccctggcgccctgctccaggagcacctccgagagcacagccgccctgggctgcctggtcaaggactacttccccgaaccggtgacggtgtcgtggaactcaggcgccctgaccagcggcgtgcacaccttcccggctgtcctacagtcctcaggactctactccctcagcagcgtggtgaccgtgccctccagcagcttgggcacgaagacctacacctgcaacgtagatcacaagcccagcaacaccaaggtggacaagagagttgagtccaaatatggtcccccatgcccaccgtgcccagcacctgagttcctggggggaccatcagtcttcctgttccccccaaaacccaaggacactctcatgatctcccggacccctgaggtcacgtgcgtggtggtggacgtgagccaggaagaccccgaggtccagttcaactggtacgtggatggcgtggaggtgcataatgccaagacaaagccgcgggaggagcagttcaacagcacgtaccgtgtggtcagcgtcctcaccgtcctgcaccaggactggctgaacggcaaggagtacaagtgcaaggtgtccaacaaaggcctcccgtcctccatcgagaaaaccatctccaaagccaaagggcagccccgagagccacaggtgtacaccctgcccccatcccaggaggagatgaccaagaaccaggtcagcctgacctgcctggtcaaaggcttctaccccagcgacatcgccgtggagtgggagagcaatgggcagccggagaacaactacaagaccacgcctcccgtgctggactccgacggctccttcttcctctacagcaggctaaccgtggacaagagcaggtggcaggaggggaatgtcttctcatgctccgtgatgcatgaggctctgcacaaccactacacacagaagagcctctccctgtctctgggtaaa

SEQ ID NO: 66 - protein, 107 aa, synthetic construct
  REGION 1..107: note = source = /note="Description of Artificial Sequence: Synthetic polypeptide"
DVVMTQSPLSLPVTLGQPASISCKASQDVGTAVAWYQQKPGQAPRLLIYWASTRHTGVPSRFSGSGSGTEFTLTISSLQPDDFATYYCQQYNSYPLTFGQGTKVEIK

SEQ ID NO: 67 - DNA, 321 bp, synthetic construct
  misc_feature 1..321: note = source = /note="Description of Artificial Sequence: Synthetic polynucleotide"
  source 1..321: mol_type = other DNA
gatgttgtgatgactcagtctccactctccctgcccgtcacccttggacagccggcctccatctcctgcaaggccagtcaggatgtgggtactgctgtagcctggtaccagcagaaacctggccaggctcccaggctcctcatctattgggcatccacccggcacactggggtcccatcaaggttcagcggcagtggatctgggacagaattcactctcaccatcagcagcctgcagcctgatgattttgcaacttattactgtcagcagtataacagctatcctctcacgttcggccaagggaccaaggtggaaatcaaa

SEQ ID NO: 68 - protein, 214 aa, synthetic construct
  REGION 1..214: note = source = /note="Description of Artificial Sequence: Synthetic polypeptide"
DVVMTQSPLSLPVTLGQPASISCKASQDVGTAVAWYQQKPGQAPRLLIYWASTRHTGVPSRFSGSGSGTEFTLTISSLQPDDFATYYCQQYNSYPLTFGQGTKVEIKRTVAAPSVFIFPPSDEQLKSGTASVVCLLNNFYPREAKVQWKVDNALQSGNSQESVTEQDSKDSTYSLSSTLTLSKADYEKHKVYACEVTHQGLSSPVTKSFNRGEC

SEQ ID NO: 69 - DNA, 642 bp, synthetic construct
  misc_feature 1..642: note = source = /note="Description of Artificial Sequence: Synthetic polynucleotide"
  source 1..642: mol_type = other DNA
gatgttgtgatgactcagtctccactctccctgcccgtcacccttggacagccggcctccatctcctgcaaggccagtcaggatgtgggtactgctgtagcctggtaccagcagaaacctggccaggctcccaggctcctcatctattgggcatccacccggcacactggggtcccatcaaggttcagcggcagtggatctgggacagaattcactctcaccatcagcagcctgcagcctgatgattttgcaacttattactgtcagcagtataacagctatcctctcacgttcggccaagggaccaaggtggaaatcaaacgtacggtggctgcaccatctgtcttcatcttcccgccatctgatgagcagttgaaatctggaactgcctctgttgtgtgcctgctgaataacttctatcccagagaggccaaagtacagtggaaggtggataacgccctccaatcgggtaactcccaggagagtgtcacagagcaggacagcaaggacagcacctacagcctcagcagcaccctgacgctgagcaaagcagactacgagaaacacaaagtctacgcctgcgaagtcacccatcagggcctgagctcgcccgtcacaaagagcttcaacaggggagagtgt

SEQ ID NO: 70 - protein, 120 aa, synthetic construct
  REGION 1..120: note = source = /note="Description of Artificial Sequence: Synthetic polypeptide"
QITLKESGPTLVKPTQTLTLTCTFSGYTFTSYWMYWVRQAPGKGLEWVSRIDPNSGSTKYNEKFKNRVTITADKSTSTAYMELSSLRSEDTAVYYCARDYRKGLYAMDYWGQGTTVTVSS

SEQ ID NO: 71 - DNA, 360 bp, synthetic construct
  misc_feature 1..360: note = source = /note="Description of Artificial Sequence: Synthetic polynucleotide"
  source 1..360: mol_type = other DNA
cagatcaccttgaaggagtctggtcctacgctggtgaaacccacacagaccctcacgctgacctgcaccttctctggctacaccttcaccagttactggatgtactgggtccgccaggctccagggaaggggctggagtgggtcagtaggattgatcctaatagtgggagtactaagtacaatgagaagttcaagaacagagtcacgattaccgcggacaaatccacgagcacagcctacatggagctgagcagcctgagatctgaggacacggccgtgtattactgtgcaagggactatagaaaggggctctatgctatggactactggggccagggcaccaccgtgaccgtgtcctcc

SEQ ID NO: 72 - protein, 447 aa, synthetic construct
  REGION 1..447: note = source = /note="Description of Artificial Sequence: Synthetic polypeptide"
QITLKESGPTLVKPTQTLTLTCTFSGYTFTSYWMYWVRQAPGKGLEWVSRIDPNSGSTKYNEKFKNRVTITADKSTSTAYMELSSLRSEDTAVYYCARDYRKGLYAMDYWGQGTTVTVSSASTKGPSVFPLAPCSRSTSESTAALGCLVKDYFPEPVTVSWNSGALTSGVHTFPAVLQSSGLYSLSSVVTVPSSSLGTKTYTCNVDHKPSNTKVDKRVESKYGPPCPPCPAPEFLGGPSVFLFPPKPKDTLMISRTPEVTCVVVDVSQEDPEVQFNWYVDGVEVHNAKTKPREEQFNSTYRVVSVLTVLHQDWLNGKEYKCKVSNKGLPSSIEKTISKAKGQPREPQVYTLPPSQEEMTKNQVSLTCLVKGFYPSDIAVEWESNGQPENNYKTTPPVLDSDGSFFLYSRLTVDKSRWQEGNVFSCSVMHEALHNHYTQKSLSLSLGK

SEQ ID NO: 73 - DNA, 1341 bp, synthetic construct
  misc_feature 1..1341: note = source = /note="Description of Artificial Sequence: Synthetic polynucleotide"
  source 1..1341: mol_type = other DNA
cagatcaccttgaaggagtctggtcctacgctggtgaaacccacacagaccctcacgctgacctgcaccttctctggctacaccttcaccagttactggatgtactgggtccgccaggctccagggaaggggctggagtgggtcagtaggattgatcctaatagtgggagtactaagtacaatgagaagttcaagaacagagtcacgattaccgcggacaaatccacgagcacagcctacatggagctgagcagcctgagatctgaggacacggccgtgtattactgtgcaagggactatagaaaggggctctatgctatggactactggggccagggcaccaccgtgaccgtgtcctccgcttccaccaagggcccatccgtcttccccctggcgccctgctccaggagcacctccgagagcacagccgccctgggctgcctggtcaaggactacttccccgaaccggtgacggtgtcgtggaactcaggcgccctgaccagcggcgtgcacaccttcccggctgtcctacagtcctcaggactctactccctcagcagcgtggtgaccgtgccctccagcagcttgggcacgaagacctacacctgcaacgtagatcacaagcccagcaacaccaaggtggacaagagagttgagtccaaatatggtcccccatgcccaccgtgcccagcacctgagttcctggggggaccatcagtcttcctgttccccccaaaacccaaggacactctcatgatctcccggacccctgaggtcacgtgcgtggtggtggacgtgagccaggaagaccccgaggtccagttcaactggtacgtggatggcgtggaggtgcataatgccaagacaaagccgcgggaggagcagttcaacagcacgtaccgtgtggtcagcgtcctcaccgtcctgcaccaggactggctgaacggcaaggagtacaagtgcaaggtgtccaacaaaggcctcccgtcctccatcgagaaaaccatctccaaagccaaagggcagccccgagagccacaggtgtacaccctgcccccatcccaggaggagatgaccaagaaccaggtcagcctgacctgcctggtcaaaggcttctaccccagcgacatcgccgtggagtgggagagcaatgggcagccggagaacaactacaagaccacgcctcccgtgctggactccgacggctccttcttcctctacagcaggctaaccgtggacaagagcaggtggcaggaggggaatgtcttctcatgctccgtgatgcatgaggctctgcacaaccactacacacagaagagcctctccctgtctctgggtaaa

SEQ ID NO: 74 - protein, 107 aa, synthetic construct
  REGION 1..107: note = source = /note="Description of Artificial Sequence: Synthetic polypeptide"
DIQMTQSPSSLSASVGDRVTITCKASQDVGTAVAWYQQKPGQAPRLLIYWASTRHTGVPSRFSGSGSGTDFTFTISSLQPEDIATYYCQQYNSYPLTFGQGTKVEIK

SEQ ID NO: 75 - DNA, 321 bp, synthetic construct
  misc_feature 1..321: note = source = /note="Description of Artificial Sequence: Synthetic polynucleotide"
  source 1..321: mol_type = other DNA
gacatccagatgacccagtctccatcctccctgtctgcatctgtaggagacagagtcaccatcacttgcaaggccagtcaggatgtgggtactgctgtagcctggtaccagcagaaacctggccaggctcccaggctcctcatctattgggcatccacccggcacactggggtcccatcaaggttcagtggaagtggatctgggacagattttactttcaccatcagcagcctgcagcctgaagatattgcaacatattactgtcagcagtataacagctatcctctcacgttcggccaagggaccaaggtggaaatcaaa

SEQ ID NO: 76 - protein, 214 aa, synthetic construct
  REGION 1..214: note = source = /note="Description of Artificial Sequence: Synthetic polypeptide"
DIQMTQSPSSLSASVGDRVTITCKASQDVGTAVAWYQQKPGQAPRLLIYWASTRHTGVPSRFSGSGSGTDFTFTISSLQPEDIATYYCQQYNSYPLTFGQGTKVEIKRTVAAPSVFIFPPSDEQLKSGTASVVCLLNNFYPREAKVQWKVDNALQSGNSQESVTEQDSKDSTYSLSSTLTLSKADYEKHKVYACEVTHQGLSSPVTKSFNRGEC

SEQ ID NO: 77 - DNA, 642 bp, synthetic construct
  misc_feature 1..642: note = source = /note="Description of Artificial Sequence: Synthetic polynucleotide"
  source 1..642: mol_type = other DNA
gacatccagatgacccagtctccatcctccctgtctgcatctgtaggagacagagtcaccatcacttgcaaggccagtcaggatgtgggtactgctgtagcctggtaccagcagaaacctggccaggctcccaggctcctcatctattgggcatccacccggcacactggggtcccatcaaggttcagtggaagtggatctgggacagattttactttcaccatcagcagcctgcagcctgaagatattgcaacatattactgtcagcagtataacagctatcctctcacgttcggccaagggaccaaggtggaaatcaaacgtacggtggctgcaccatctgtcttcatcttcccgccatctgatgagcagttgaaatctggaactgcctctgttgtgtgcctgctgaataacttctatcccagagaggccaaagtacagtggaaggtggataacgccctccaatcgggtaactcccaggagagtgtcacagagcaggacagcaaggacagcacctacagcctcagcagcaccctgacgctgagcaaagcagactacgagaaacacaaagtctacgcctgcgaagtcacccatcagggcctgagctcgcccgtcacaaagagcttcaacaggggagagtgt

SEQ ID NO: 78 - protein, 120 aa, synthetic construct
  REGION 1..120: note = source = /note="Description of Artificial Sequence: Synthetic polypeptide"
EVQLVQSGAEVKKPGATVKISCKVSGYTFTSYWMYWVRQARGQRLEWIGRIDPNSGSTKYNEKFKNRFTISRDNSKNTLYLQMNSLRAEDTAVYYCARDYRKGLYAMDYWGQGTTVTVSS

SEQ ID NO: 79 - DNA, 360 bp, synthetic construct
  misc_feature 1..360: note = source = /note="Description of Artificial Sequence: Synthetic polynucleotide"
  source 1..360: mol_type = other DNA
gaggtccagctggtacagtctggggctgaggtgaagaagcctggggctacagtgaaaatctcctgcaaggtttctggctacaccttcaccagttactggatgtactgggtgcgacaggctcgtggacaacgccttgagtggataggtaggattgatcctaatagtgggagtactaagtacaatgagaagttcaagaacagattcaccatctccagagacaattccaagaacacgctgtatcttcaaatgaacagcctgagagccgaggacacggccgtgtattactgtgcaagggactatagaaaggggctctatgctatggactactggggccagggcaccaccgtgaccgtgtcctcc

SEQ ID NO: 80 - protein, 446 aa, synthetic construct
  REGION 1..446: note = source = /note="Description of Artificial Sequence: Synthetic polypeptide"
EVQLVQSGAEVKKPGATVKISCKVSGYTFTSYWMYWVRQARGQRLEWIGRIDPNSGSTKYNEKFKNRFTISRDNSKNTLYLQMNSLRAEDTAVYYCARDYRKGLYAMDYWGQGTTVTVSSASTKGPSVFPLAPCSRSTSESTAALGCLVKDYFPEPVTVSWNSGALTSGVHTFPAVLQSSGLYSLSSVVTVPSSSLGTKTYTCNVDHKPSNTKVDKRVESKYGPPCPPCPAPEFLGGPSVFLFPPKPKDTLMISRTPEVTCVVVDVSQEDPEVQFNWYVDGVEVHNAKTKPREEQFNSTYRVVSVLTVLHQDWLNGKEYKCKVSNKGLPSSIEKTISKAKGQPREPQVYTLPPSQEEMTKNQVSLTCLVKGFYPSDIAVEWESNGQPENNYKTTPPVLDSDGSFFLYSRLTVDKSRWQEGNVFSCSVMHEALHNHYTQKSLSLSLG

SEQ ID NO: 81 - DNA, 1341 bp, synthetic construct
  misc_feature 1..1341: note = source = /note="Description of Artificial Sequence: Synthetic polynucleotide"
  source 1..1341: mol_type = other DNA
gaggtccagctggtacagtctggggctgaggtgaagaagcctggggctacagtgaaaatctcctgcaaggtttctggctacaccttcaccagttactggatgtactgggtgcgacaggctcgtggacaacgccttgagtggataggtaggattgatcctaatagtgggagtactaagtacaatgagaagttcaagaacagattcaccatctccagagacaattccaagaacacgctgtatcttcaaatgaacagcctgagagccgaggacacggccgtgtattactgtgcaagggactatagaaaggggctctatgctatggactactggggccagggcaccaccgtgaccgtgtcctccgcttccaccaagggcccatccgtcttccccctggcgccctgctccaggagcacctccgagagcacagccgccctgggctgcctggtcaaggactacttccccgaaccggtgacggtgtcgtggaactcaggcgccctgaccagcggcgtgcacaccttcccggctgtcctacagtcctcaggactctactccctcagcagcgtggtgaccgtgccctccagcagcttgggcacgaagacctacacctgcaacgtagatcacaagcccagcaacaccaaggtggacaagagagttgagtccaaatatggtcccccatgcccaccgtgcccagcacctgagttcctggggggaccatcagtcttcctgttccccccaaaacccaaggacactctcatgatctcccggacccctgaggtcacgtgcgtggtggtggacgtgagccaggaagaccccgaggtccagttcaactggtacgtggatggcgtggaggtgcataatgccaagacaaagccgcgggaggagcagttcaacagcacgtaccgtgtggtcagcgtcctcaccgtcctgcaccaggactggctgaacggcaaggagtacaagtgcaaggtgtccaacaaaggcctcccgtcctccatcgagaaaaccatctccaaagccaaagggcagccccgagagccacaggtgtacaccctgcccccatcccaggaggagatgaccaagaaccaggtcagcctgacctgcctggtcaaaggcttctaccccagcgacatcgccgtggagtgggagagcaatgggcagccggagaacaactacaagaccacgcctcccgtgctggactccgacggctccttcttcctctacagcaggctaaccgtggacaagagcaggtggcaggaggggaatgtcttctcatgctccgtgatgcatgaggctctgcacaaccactacacacagaagagcctctccctgtctctgggtaaa

SEQ ID NO: 82 - protein, 107 aa, synthetic construct
  REGION 1..107: note = source = /note="Description of Artificial Sequence: Synthetic polypeptide"
AIQLTQSPSSLSASVGDRVTITCKASQDVGTAVAWYLQKPGQSPQLLIYWASTRHTGVPSRFSGSGSGTDFTFTISSLEAEDAATYYCQQYNSYPLTFGQGTKVEIK

SEQ ID NO: 83 - DNA, 321 bp, synthetic construct
  misc_feature 1..321: note = source = /note="Description of Artificial Sequence: Synthetic polynucleotide"
  source 1..321: mol_type = other DNA
gccatccagttgacccagtctccatcctccctgtctgcatctgtaggagacagagtcaccatcacttgcaaggccagtcaggatgtgggtactgctgtagcctggtacctgcagaagccagggcagtctccacagctcctgatctattgggcatccacccggcacactggggtcccctcgaggttcagtggcagtggatctgggacagatttcacctttaccatcagtagcctggaagctgaagatgctgcaacatattactgtcagcagtataacagctatcctctcacgttcggccaagggaccaaggtggaaatcaaa

SEQ ID NO: 84 - protein, 214 aa, synthetic construct
  REGION 1..214: note = source = /note="Description of Artificial Sequence: Synthetic polypeptide"
AIQLTQSPSSLSASVGDRVTITCKASQDVGTAVAWYLQKPGQSPQLLIYWASTRHTGVPSRFSGSGSGTDFTFTISSLEAEDAATYYCQQYNSYPLTFGQGTKVEIKRTVAAPSVFIFPPSDEQLKSGTASVVCLLNNFYPREAKVQWKVDNALQSGNSQESVTEQDSKDSTYSLSSTLTLSKADYEKHKVYACEVTHQGLSSPVTKSFNRGEC

SEQ ID NO: 85 - DNA, 642 bp, synthetic construct
  misc_feature 1..642: note = source = /note="Description of Artificial Sequence: Synthetic polynucleotide"
  source 1..642: mol_type = other DNA
gccatccagttgacccagtctccatcctccctgtctgcatctgtaggagacagagtcaccatcacttgcaaggccagtcaggatgtgggtactgctgtagcctggtacctgcagaagccagggcagtctccacagctcctgatctattgggcatccacccggcacactggggtcccctcgaggttcagtggcagtggatctgggacagatttcacctttaccatcagtagcctggaagctgaagatgctgcaacatattactgtcagcagtataacagctatcctctcacgttcggccaagggaccaaggtggaaatcaaacgtacggtggctgcaccatctgtcttcatcttcccgccatctgatgagcagttgaaatctggaactgcctctgttgtgtgcctgctgaataacttctatcccagagaggccaaagtacagtggaaggtggataacgccctccaatcgggtaactcccaggagagtgtcacagagcaggacagcaaggacagcacctacagcctcagcagcaccctgacgctgagcaaagcagactacgagaaacacaaagtctacgcctgcgaagtcacccatcagggcctgagctcgcccgtcacaaagagcttcaacaggggagagtgt

SEQ ID NO: 86 - protein, 107 aa, synthetic construct
  REGION 1..107: note = source = /note="Description of Artificial Sequence: Synthetic polypeptide"
EIVLTQSPDFQSVTPKEKVTITCKASQDVGTAVAWYQQKPGQAPRLLIYWASTRHTGVPSRFSGSGSGTEFTLTISSLQPDDFATYYCQQYNSYPLTFGQGTKVEIK

SEQ ID NO: 87 - DNA, 321 bp, synthetic construct
  misc_feature 1..321: note = source = /note="Description of Artificial Sequence: Synthetic polynucleotide"
  source 1..321: mol_type = other DNA
gaaattgtgctgactcagtctccagactttcagtctgtgactccaaaggagaaagtcaccatcacctgcaaggccagtcaggatgtgggtactgctgtagcctggtaccagcagaaacctggccaggctcccaggctcctcatctattgggcatccacccggcacactggggtcccatcaaggttcagcggcagtggatctgggacagaattcactctcaccatcagcagcctgcagcctgatgattttgcaacttattactgtcagcagtataacagctatcctctcacgttcggccaagggaccaaggtggaaatcaaa

SEQ ID NO: 88 - protein, 214 aa, synthetic construct
  REGION 1..214: note = source = /note="Description of Artificial Sequence: Synthetic polypeptide"
EIVLTQSPDFQSVTPKEKVTITCKASQDVGTAVAWYQQKPGQAPRLLIYWASTRHTGVPSRFSGSGSGTEFTLTISSLQPDDFATYYCQQYNSYPLTFGQGTKVEIKRTVAAPSVFIFPPSDEQLKSGTASVVCLLNNFYPREAKVQWKVDNALQSGNSQESVTEQDSKDSTYSLSSTLTLSKADYEKHKVYACEVTHQGLSSPVTKSFNRGEC

SEQ ID NO: 89 - DNA, 642 bp, synthetic construct
  misc_feature 1..642: note = source = /note="Description of Artificial Sequence: Synthetic polynucleotide"
  source 1..642: mol_type = other DNA
gaaattgtgctgactcagtctccagactttcagtctgtgactccaaaggagaaagtcaccatcacctgcaaggccagtcaggatgtgggtactgctgtagcctggtaccagcagaaacctggccaggctcccaggctcctcatctattgggcatccacccggcacactggggtcccatcaaggttcagcggcagtggatctgggacagaattcactctcaccatcagcagcctgcagcctgatgattttgcaacttattactgtcagcagtataacagctatcctctcacgttcggccaagggaccaaggtggaaatcaaacgtacggtggctgcaccatctgtcttcatcttcccgccatctgatgagcagttgaaatctggaactgcctctgttgtgtgcctgctgaataacttctatcccagagaggccaaagtacagtggaaggtggataacgccctccaatcgggtaactcccaggagagtgtcacagagcaggacagcaaggacagcacctacagcctcagcagcaccctgacgctgagcaaagcagactacgagaaacacaaagtctacgcctgcgaagtcacccatcagggcctgagctcgcccgtcacaaagagcttcaacaggggagagtgt

SEQ ID NO: 90 - DNA, 360 bp, synthetic construct
  misc_feature 1..360: note = source = /note="Description of Artificial Sequence: Synthetic polynucleotide"
  source 1..360: mol_type = other DNA
gaagtgcagctggtgcagtcaggcgccgaagtgaagaagcccggcgagtcactgagaattagctgtaaaggttcaggctacaccttcactagctactggatgtactgggtccgacaggccccagggcaaggcctggagtggatgggtagaatcgaccctaatagcggctctactaagtataacgagaagtttaagaatagagtgactattagcgtggacacctctaagaatcagtttagcctgaagctgtctagcgtgaccgccgctgacaccgccgtctactactgcgctagagactatagaaagggcctgtacgctatggactactggggtcaaggcactaccgtgaccgtgtcttca

SEQ ID NO: 91 - protein, 446 aa, synthetic construct
  REGION 1..446: note = source = /note="Description of Artificial Sequence: Synthetic polypeptide"
EVQLVQSGAEVKKPGESLRISCKGSGYTFTSYWMYWVRQAPGQGLEWMGRIDPNSGSTKYNEKFKNRVTISVDTSKNQFSLKLSSVTAADTAVYYCARDYRKGLYAMDYWGQGTTVTVSSASTKGPSVFPLAPCSRSTSESTAALGCLVKDYFPEPVTVSWNSGALTSGVHTFPAVLQSSGLYSLSSVVTVPSSSLGTKTYTCNVDHKPSNTKVDKRVESKYGPPCPPCPAPEFLGGPSVFLFPPKPKDTLMISRTPEVTCVVVDVSQEDPEVQFNWYVDGVEVHNAKTKPREEQFNSTYRVVSVLTVLHQDWLNGKEYKCKVSNKGLPSSIEKTISKAKGQPREPQVYTLPPSQEEMTKNQVSLTCLVKGFYPSDIAVEWESNGQPENNYKTTPPVLDSDGSFFLYSRLTVDKSRWQEGNVFSCSVMHEALHNHYTQKSLSLSLG

SEQ ID NO: 92 - DNA, 1338 bp, synthetic construct
  misc_feature 1..1338: note = source = /note="Description of Artificial Sequence: Synthetic polynucleotide"
  source 1..1338: mol_type = other DNA
gaagtgcagctggtgcagtcaggcgccgaagtgaagaagcccggcgagtcactgagaattagctgtaaaggttcaggctacaccttcactagctactggatgtactgggtccgacaggccccagggcaaggcctggagtggatgggtagaatcgaccctaatagcggctctactaagtataacgagaagtttaagaatagagtgactattagcgtggacacctctaagaatcagtttagcctgaagctgtctagcgtgaccgccgctgacaccgccgtctactactgcgctagagactatagaaagggcctgtacgctatggactactggggtcaaggcactaccgtgaccgtgtcttcagctagcactaagggcccgtccgtgttccccctggcaccttgtagccggagcactagcgaatccaccgctgccctcggctgcctggtcaaggattacttcccggagcccgtgaccgtgtcctggaacagcggagccctgacctccggagtgcacaccttccccgctgtgctgcagagctccgggctgtactcgctgtcgtcggtggtcacggtgccttcatctagcctgggtaccaagacctacacttgcaacgtggaccacaagccttccaacactaaggtggacaagcgcgtcgaatcgaagtacggcccaccgtgcccgccttgtcccgcgccggagttcctcggcggtccctcggtctttctgttcccaccgaagcccaaggacactttgatgatttcccgcacccctgaagtgacatgcgtggtcgtggacgtgtcacaggaagatccggaggtgcagttcaattggtacgtggatggcgtcgaggtgcacaacgccaaaaccaagccgagggaggagcagttcaactccacttaccgcgtcgtgtccgtgctgacggtgctgcatcaggactggctgaacgggaaggagtacaagtgcaaagtgtccaacaagggacttcctagctcaatcgaaaagaccatctcgaaagccaagggacagccccgggaaccccaagtgtataccctgccaccgagccaggaagaaatgactaagaaccaagtctcattgacttgccttgtgaagggcttctacccatcggatatcgccgtggaatgggagtccaacggccagccggaaaacaactacaagaccacccctccggtgctggactcagacggatccttcttcctctactcgcggctgaccgtggataagagcagatggcaggagggaaatgtgttcagctgttctgtgatgcatgaagccctgcacaaccactacactcagaagtccctgtccctctccctggga

SEQ ID NO: 93 - DNA, 321 bp, synthetic construct
  misc_feature 1..321: note = source = /note="Description of Artificial Sequence: Synthetic polynucleotide"
  source 1..321: mol_type = other DNA
gagatcgtcctgactcagtcacccgactttcagtcagtgacccctaaagagaaagtcactatcacctgtaaagcctctcaggacgtgggcaccgccgtggcctggtatctgcagaagcctggtcaatcacctcagctgctgatctactgggcctctactagacacaccggcgtgccctctaggtttagcggtagcggtagtggcaccgacttcaccttcactatctcttcactgcagcccgaggatatcgctacctactactgtcagcagtataatagctaccccctgaccttcggtcaaggcactaaggtcgagattaag

SEQ ID NO: 94 - DNA, 642 bp, synthetic construct
  misc_feature 1..642: note = source = /note="Description of Artificial Sequence: Synthetic polynucleotide"
  source 1..642: mol_type = other DNA
gagatcgtcctgactcagtcacccgactttcagtcagtgacccctaaagagaaagtcactatcacctgtaaagcctctcaggacgtgggcaccgccgtggcctggtatctgcagaagcctggtcaatcacctcagctgctgatctactgggcctctactagacacaccggcgtgccctctaggtttagcggtagcggtagtggcaccgacttcaccttcactatctcttcactgcagcccgaggatatcgctacctactactgtcagcagtataatagctaccccctgaccttcggtcaaggcactaaggtcgagattaagcgtacggtggccgctcccagcgtgttcatcttcccccccagcgacgagcagctgaagagcggcaccgccagcgtggtgtgcctgctgaacaacttctacccccgggaggccaaggtgcagtggaaggtggacaacgccctgcagagcggcaacagccaggagagcgtcaccgagcaggacagcaaggactccacctacagcctgagcagcaccctgaccctgagcaaggccgactacgagaagcataaggtgtacgcctgcgaggtgacccaccagggcctgtccagccccgtgaccaagagcttcaacaggggcgagtgc

SEQ ID NO: 95 - DNA, 360 bp, synthetic construct
  misc_feature 1..360: note = source = /note="Description of Artificial Sequence: Synthetic polynucleotide"
  source 1..360: mol_type = other DNA
gaagtgcagctggtgcagtcaggcgccgaagtgaagaaacccggcgctaccgtgaagattagctgtaaagtctcaggctacaccttcactagctactggatgtactgggtccgacaggctaccggtcaaggcctggagtggatgggtagaatcgaccctaatagcggctctactaagtataacgagaagtttaagaatagagtgactatcaccgccgataagtctactagcaccgcctatatggaactgtctagcctgagatcagaggacaccgccgtctactactgcgctagagactatagaaagggcctgtacgctatggactactggggtcaaggcactaccgtgaccgtgtcttca

SEQ ID NO: 96 - protein, 446 aa, synthetic construct
  REGION 1..446: note = source = /note="Description of Artificial Sequence: Synthetic polypeptide"
EVQLVQSGAEVKKPGATVKISCKVSGYTFTSYWMYWVRQATGQGLEWMGRIDPNSGSTKYNEKFKNRVTITADKSTSTAYMELSSLRSEDTAVYYCARDYRKGLYAMDYWGQGTTVTVSSASTKGPSVFPLAPCSRSTSESTAALGCLVKDYFPEPVTVSWNSGALTSGVHTFPAVLQSSGLYSLSSVVTVPSSSLGTKTYTCNVDHKPSNTKVDKRVESKYGPPCPPCPAPEFLGGPSVFLFPPKPKDTLMISRTPEVTCVVVDVSQEDPEVQFNWYVDGVEVHNAKTKPREEQFNSTYRVVSVLTVLHQDWLNGKEYKCKVSNKGLPSSIEKTISKAKGQPREPQVYTLPPSQEEMTKNQVSLTCLVKGFYPSDIAVEWESNGQPENNYKTTPPVLDSDGSFFLYSRLTVDKSRWQEGNVFSCSVMHEALHNHYTQKSLSLSLG

SEQ ID NO: 97 - DNA, 1338 bp, synthetic construct
  misc_feature 1..1338: note = source = /note="Description of Artificial Sequence: Synthetic polynucleotide"
  source 1..1338: mol_type = other DNA
gaagtgcagctggtgcagtcaggcgccgaagtgaagaaacccggcgctaccgtgaagattagctgtaaagtctcaggctacaccttcactagctactggatgtactgggtccgacaggctaccggtcaaggcctggagtggatgggtagaatcgaccctaatagcggctctactaagtataacgagaagtttaagaatagagtgactatcaccgccgataagtctactagcaccgcctatatggaactgtctagcctgagatcagaggacaccgccgtctactactgcgctagagactatagaaagggcctgtacgctatggactactggggtcaaggcactaccgtgaccgtgtcttcagctagcactaagggcccgtccgtgttccccctggcaccttgtagccggagcactagcgaatccaccgctgccctcggctgcctggtcaaggattacttcccggagcccgtgaccgtgtcctggaacagcggagccctgacctccggagtgcacaccttccccgctgtgctgcagagctccgggctgtactcgctgtcgtcggtggtcacggtgccttcatctagcctgggtaccaagacctacacttgcaacgtggaccacaagccttccaacactaaggtggacaagcgcgtcgaatcgaagtacggcccaccgtgcccgccttgtcccgcgccggagttcctcggcggtccctcggtctttctgttcccaccgaagcccaaggacactttgatgatttcccgcacccctgaagtgacatgcgtggtcgtggacgtgtcacaggaagatccggaggtgcagttcaattggtacgtggatggcgtcgaggtgcacaacgccaaaaccaagccgagggaggagcagttcaactccacttaccgcgtcgtgtccgtgctgacggtgctgcatcaggactggctgaacgggaaggagtacaagtgcaaagtgtccaacaagggacttcctagctcaatcgaaaagaccatctcgaaagccaagggacagccccgggaaccccaagtgtataccctgccaccgagccaggaagaaatgactaagaaccaagtctcattgacttgccttgtgaagggcttctacccatcggatatcgccgtggaatgggagtccaacggccagccggaaaacaactacaagaccacccctccggtgctggactcagacggatccttcttcctctactcgcggctgaccgtggataagagcagatggcaggagggaaatgtgttcagctgttctgtgatgcatgaagccctgcacaaccactacactcagaagtccctgtccctctccctggga

SEQ ID NO: 98 - DNA, 321 bp, synthetic construct
  misc_feature 1..321: note = source = /note="Description of Artificial Sequence: Synthetic polynucleotide"
  source 1..321: mol_type = other DNA
gacgtcgtgatgactcagtcacccctgagcctgcccgtgaccctggggcagcccgcctctattagctgtaaagcctctcaggacgtgggcaccgccgtggcctggtatcagcagaagccagggcaagcccctagactgctgatctactgggcctctactagacacaccggcgtgccctctaggtttagcggtagcggtagtggcaccgagttcaccctgactatctcttcactgcagcccgacgacttcgctacctactactgtcagcagtataatagctaccccctgaccttcggtcaaggcactaaggtcgagattaag

SEQ ID NO: 99 - DNA, 642 bp, synthetic construct
  misc_feature 1..642: note = source = /note="Description of Artificial Sequence: Synthetic polynucleotide"
  source 1..642: mol_type = other DNA
gacgtcgtgatgactcagtcacccctgagcctgcccgtgaccctggggcagcccgcctctattagctgtaaagcctctcaggacgtgggcaccgccgtggcctggtatcagcagaagccagggcaagcccctagactgctgatctactgggcctctactagacacaccggcgtgccctctaggtttagcggtagcggtagtggcaccgagttcaccctgactatctcttcactgcagcccgacgacttcgctacctactactgtcagcagtataatagctaccccctgaccttcggtcaaggcactaaggtcgagattaagcgtacggtggccgctcccagcgtgttcatcttcccccccagcgacgagcagctgaagagcggcaccgccagcgtggtgtgcctgctgaacaacttctacccccgggaggccaaggtgcagtggaaggtggacaacgccctgcagagcggcaacagccaggagagcgtcaccgagcaggacagcaaggactccacctacagcctgagcagcaccctgaccctgagcaaggccgactacgagaagcataaggtgtacgcctgcgaggtgacccaccagggcctgtccagccccgtgaccaagagcttcaacaggggcgagtgc

SEQ ID NO: 100 - DNA, 360 bp, synthetic construct
  misc_feature 1..360: note = source = /note="Description of Artificial Sequence: Synthetic polynucleotide"
  source 1..360: mol_type = other DNA
gaagtgcagctggtgcagtcaggcgccgaagtgaagaaacccggcgctaccgtgaagattagctgtaaagtctcaggctacaccttcactagctactggatgtactgggtccgacaggctagagggcaaagactggagtggatcggtagaatcgaccctaatagcggctctactaagtataacgagaagtttaagaataggttcactattagtagggataactctaagaacaccctgtacctgcagatgaatagcctgagagccgaggacaccgccgtctactactgcgctagagactatagaaagggcctgtacgctatggactactggggtcaaggcactaccgtgaccgtgtcttca

SEQ ID NO: 101 - DNA, 1338 bp, synthetic construct
  misc_feature 1..1338: note = source = /note="Description of Artificial Sequence: Synthetic polynucleotide"
  source 1..1338: mol_type = other DNA
gaagtgcagctggtgcagtcaggcgccgaagtgaagaaacccggcgctaccgtgaagattagctgtaaagtctcaggctacaccttcactagctactggatgtactgggtccgacaggctagagggcaaagactggagtggatcggtagaatcgaccctaatagcggctctactaagtataacgagaagtttaagaataggttcactattagtagggataactctaagaacaccctgtacctgcagatgaatagcctgagagccgaggacaccgccgtctactactgcgctagagactatagaaagggcctgtacgctatggactactggggtcaaggcactaccgtgaccgtgtcttcagctagcactaagggcccgtccgtgttccccctggcaccttgtagccggagcactagcgaatccaccgctgccctcggctgcctggtcaaggattacttcccggagcccgtgaccgtgtcctggaacagcggagccctgacctccggagtgcacaccttccccgctgtgctgcagagctccgggctgtactcgctgtcgtcggtggtcacggtgccttcatctagcctgggtaccaagacctacacttgcaacgtggaccacaagccttccaacactaaggtggacaagcgcgtcgaatcgaagtacggcccaccgtgcccgccttgtcccgcgccggagttcctcggcggtccctcggtctttctgttcccaccgaagcccaaggacactttgatgatttcccgcacccctgaagtgacatgcgtggtcgtggacgtgtcacaggaagatccggaggtgcagttcaattggtacgtggatggcgtcgaggtgcacaacgccaaaaccaagccgagggaggagcagttcaactccacttaccgcgtcgtgtccgtgctgacggtgctgcatcaggactggctgaacgggaaggagtacaagtgcaaagtgtccaacaagggacttcctagctcaatcgaaaagaccatctcgaaagccaagggacagccccgggaaccccaagtgtataccctgccaccgagccaggaagaaatgactaagaaccaagtctcattgacttgccttgtgaagggcttctacccatcggatatcgccgtggaatgggagtccaacggccagccggaaaacaactacaagaccacccctccggtgctggactcagacggatccttcttcctctactcgcggctgaccgtggataagagcagatggcaggagggaaatgtgttcagctgttctgtgatgcatgaagccctgcacaaccactacactcagaagtccctgtccctctccctggga

SEQ ID NO: 102 - DNA, 321 bp, synthetic construct
  misc_feature 1..321: note = source = /note="Description of Artificial Sequence: Synthetic polynucleotide"
  source 1..321: mol_type = other DNA
gctattcagctgactcagtcacctagtagcctgagcgctagtgtgggcgatagagtgactatcacctgtaaagcctctcaggacgtgggcaccgccgtggcctggtatctgcagaagcctggtcaatcacctcagctgctgatctactgggcctctactagacacaccggcgtgccctctaggtttagcggtagcggtagtggcaccgacttcaccttcactatctcttcactggaagccgaggacgccgctacctactactgtcagcagtataatagctaccccctgaccttcggtcaaggcactaaggtcgagattaag

SEQ ID NO: 103 - DNA, 642 bp, synthetic construct
  misc_feature 1..642: note = source = /note="Description of Artificial Sequence: Synthetic polynucleotide"
  source 1..642: mol_type = other DNA
gctattcagctgactcagtcacctagtagcctgagcgctagtgtgggcgatagagtgactatcacctgtaaagcctctcaggacgtgggcaccgccgtggcctggtatctgcagaagcctggtcaatcacctcagctgctgatctactgggcctctactagacacaccggcgtgccctctaggtttagcggtagcggtagtggcaccgacttcaccttcactatctcttcactggaagccgaggacgccgctacctactactgtcagcagtataatagctaccccctgaccttcggtcaaggcactaaggtcgagattaagcgtacggtggccgctcccagcgtgttcatcttcccccccagcgacgagcagctgaagagcggcaccgccagcgtggtgtgcctgctgaacaacttctacccccgggaggccaaggtgcagtggaaggtggacaacgccctgcagagcggcaacagccaggagagcgtcaccgagcaggacagcaaggactccacctacagcctgagcagcaccctgaccctgagcaaggccgactacgagaagcataaggtgtacgcctgcgaggtgacccaccagggcctgtccagccccgtgaccaagagcttcaacaggggcgagtgc

SEQ ID NO: 104 - DNA, 15 bp, synthetic construct
  misc_feature 1..15: note = source = /note="Description of Artificial Sequence: Synthetic oligonucleotide"
  source 1..15: mol_type = other DNA
agttactggatgtac

SEQ ID NO: 105 - DNA, 51 bp, synthetic construct
  misc_feature 1..51: note = source = /note="Description of Artificial Sequence: Synthetic oligonucleotide"
  source 1..51: mol_type = other DNA
aggattgatcctaatagtgggagtactaagtacaatgagaagttcaagaac

SEQ ID NO: 106 - DNA, 33 bp, synthetic construct
  misc_feature 1..33: note = source = /note="Description of Artificial Sequence: Synthetic oligonucleotide"
  source 1..33: mol_type = other DNA
gactatagaaaggggctctatgctatggactac

SEQ ID NO: 107 - DNA, 21 bp, synthetic construct
  misc_feature 1..21: note = source = /note="Description of Artificial Sequence: Synthetic oligonucleotide"
  source 1..21: mol_type = other DNA
ggctacaccttcaccagttac

SEQ ID NO: 108 - DNA, 18 bp, synthetic construct
  misc_feature 1..18: note = source = /note="Description of Artificial Sequence: Synthetic oligonucleotide"
  source 1..18: mol_type = other DNA
gatcctaatagtgggagt

SEQ ID NO: 109 - DNA, 27 bp, synthetic construct
  misc_feature 1..27: note = source = /note="Description of Artificial Sequence: Synthetic oligonucleotide"
  source 1..27: mol_type = other DNA
cagcagtataacagctatcctctcacg

SEQ ID NO: 110 - DNA, 21 bp, synthetic construct
  misc_feature 1..21: note = source = /note="Description of Artificial Sequence: Synthetic oligonucleotide"
  source 1..21: mol_type = other DNA
agtcaggatgtgggtactgct

SEQ ID NO: 111 - skipped

SEQ ID NO: 112 - DNA, 18 bp, synthetic construct
  misc_feature 1..18: note = source = /note="Description of Artificial Sequence: Synthetic oligonucleotide"
  source 1..18: mol_type = other DNA
tataacagctatcctctc

SEQ ID NO: 113 - DNA, 15 bp, synthetic construct
  misc_feature 1..15: note = source = /note="Description of Artificial Sequence: Synthetic oligonucleotide"
  source 1..15: mol_type = other DNA
agctactggatgtac

SEQ ID NO: 114 - DNA, 51 bp, synthetic construct
  misc_feature 1..51: note = source = /note="Description of Artificial Sequence: Synthetic oligonucleotide"
  source 1..51: mol_type = other DNA
agaatcgaccctaatagcggctctactaagtataacgagaagtttaagaat

SEQ ID NO: 115 - DNA, 33 bp, synthetic construct
  misc_feature 1..33: note = source = /note="Description of Artificial Sequence: Synthetic oligonucleotide"
  source 1..33: mol_type = other DNA
gactatagaaagggcctgtacgctatggactac

SEQ ID NO: 116 - DNA, 21 bp, synthetic construct
  misc_feature 1..21: note = source = /note="Description of Artificial Sequence: Synthetic oligonucleotide"
  source 1..21: mol_type = other DNA
ggctacaccttcactagctac

SEQ ID NO: 117 - DNA, 18 bp, synthetic construct
  misc_feature 1..18: note = source = /note="Description of Artificial Sequence: Synthetic oligonucleotide"
  source 1..18: mol_type = other DNA
gaccctaatagcggctct

SEQ ID NO: 118 - DNA, 33 bp, synthetic construct
  misc_feature 1..33: note = source = /note="Description of Artificial Sequence: Synthetic oligonucleotide"
  source 1..33: mol_type = other DNA
aaagcctctcaggacgtgggcaccgccgtggcc

SEQ ID NO: 119 - DNA, 21 bp, synthetic construct
  misc_feature 1..21: note = source = /note="Description of Artificial Sequence: Synthetic oligonucleotide"
  source 1..21: mol_type = other DNA
tgggcctctactagacacacc

SEQ ID NO: 120 - DNA, 27 bp, synthetic construct
  misc_feature 1..27: note = source = /note="Description of Artificial Sequence: Synthetic oligonucleotide"
  source 1..27: mol_type = other DNA
cagcagtataatagctaccccctgacc

SEQ ID NO: 121 - DNA, 21 bp, synthetic construct
  misc_feature 1..21: note = source = /note="Description of Artificial Sequence: Synthetic oligonucleotide"
  source 1..21: mol_type = other DNA
tctcaggacgtgggcaccgcc

SEQ ID NO: 122 - skipped

SEQ ID NO: 123 - DNA, 18 bp, synthetic construct
  misc_feature 1..18: note = source = /note="Description of Artificial Sequence: Synthetic oligonucleotide"
  source 1..18: mol_type = other DNA
tataatagctaccccctg

SEQ ID NO: 124 - protein, 25 aa, synthetic construct [sequence omitted]

SEQ ID NO: 125 - DNA, 75 bp, synthetic construct
  misc_feature 1..75: note = source = /note="Description of Artificial Sequence: Synthetic oligonucleotide"
  source 1..75: mol_type = other DNA
caggttcagctggtgcagtctggagctgaggtgaagaagcctggggcctcagtgaaggtctcctgcaaggcttct

SEQ ID NO: 126 - protein, 25 aa, synthetic construct
  REGION 1..25: note = source = /note="Description of Artificial Sequence: Synthetic peptide"
EVQLVQSGAEVKKPGESLRISCKGS

SEQ ID NO: 127 - DNA, 75 bp, synthetic construct
  misc_feature 1..75: note = source = /note="Description of Artificial Sequence: Synthetic oligonucleotide"
  source 1..75: mol_type = other DNA
gaagtgcagctggtgcagtctggagcagaggtgaaaaagcccggggagtctctgaggatctcctgtaagggttct

SEQ ID NO: 128 - protein, 25 aa, synthetic construct
  REGION 1..25: note = source = /note="Description of Artificial Sequence: Synthetic peptide"
EVQLVQSGAEVKKPGATVKISCKVS

SEQ ID NO: 129 - DNA, 75 bp, synthetic construct
  misc_feature 1..75: note = source = /note="Description of Artificial Sequence: Synthetic oligonucleotide"
  source 1..75: mol_type = other DNA
gaggtccagctggtacagtctggggctgaggtgaagaagcctggggctacagtgaaaatctcctgcaaggtttct

SEQ ID NO: 130 - protein, 25 aa, synthetic construct
  REGION 1..25: note = source = /note="Description of Artificial Sequence: Synthetic peptide"
QITLKESGPTLVKPTQTLTLTCTFS

SEQ ID NO: 131 - DNA, 75 bp, synthetic construct
  misc_feature 1..75: note = source = /note="Description of Artificial Sequence: Synthetic oligonucleotide"
  source 1..75: mol_type = other DNA
cagatcaccttgaaggagtctggtcctacgctggtgaaacccacacagaccctcacgctgacctgcaccttctct

SEQ ID NO: 132 - protein, 14 aa, synthetic construct
  REGION 1..14: note = source = /note="Description of Artificial Sequence: Synthetic peptide"
WVRQATGQGLEWMG

SEQ ID NO: 133 - DNA, 42 bp, synthetic construct
  misc_feature 1..42: note = source = /note="Description of Artificial Sequence: Synthetic oligonucleotide"
  source 1..42: mol_type = other DNA
tgggtgcgacaggccactggacaagggcttgagtggatgggt

SEQ ID NO: 134 - protein, 14 aa, synthetic construct
  REGION 1..14: note = source = /note="Description of Artificial Sequence: Synthetic peptide"
WVRQAPGQGLEWMG

SEQ ID NO: 135 - DNA, 42 bp, synthetic construct
  misc_feature 1..42: note = source = /note="Description of Artificial Sequence: Synthetic oligonucleotide"
  source 1..42: mol_type = other DNA
tgggtgcgacaggcccctggacaagggcttgagtggatgggt

SEQ ID NO: 136 - protein, 14 aa, synthetic construct
  REGION 1..14: note = source = /note="Description of Artificial Sequence: Synthetic peptide"
WIRQPPGKGLEWIG

SEQ ID NO: 137 - DNA, 42 bp, synthetic construct
  misc_feature 1..42: note = source = /note="Description of Artificial Sequence: Synthetic oligonucleotide"
  source 1..42: mol_type = other DNA
tggatccgccagcccccagggaaggggctggagtggattggt

SEQ ID NO: 138 - protein, 14 aa, synthetic construct
  REGION 1..14: note = source = /note="Description of Artificial Sequence: Synthetic peptide"
WIRQSPSRGLEWLG

SEQ ID NO: 139 - DNA, 42 bp, synthetic construct
  misc_feature 1..42: note = source = /note="Description of Artificial Sequence: Synthetic oligonucleotide"
  source 1..42: mol_type = other DNA
tggatcaggcagtccccatcgagaggccttgagtggctgggt

SEQ ID NO: 140 - protein, 14 aa, synthetic construct
  REGION 1..14: note = source = /note="Description of Artificial Sequence: Synthetic peptide"
WVRQARGQRLEWIG

SEQ ID NO: 141 - DNA, 42 bp, synthetic construct
  misc_feature 1..42: note = source = /note="Description of Artificial Sequence: Synthetic oligonucleotide"
  source 1..42: mol_type = other DNA
tgggtgcgacaggctcgtggacaacgccttgagtggataggt

SEQ ID NO: 142 - protein, 14 aa, synthetic construct
  REGION 1..14: note = source = /note="Description of Artificial Sequence: Synthetic peptide"
WVRQAPGKGLEWVS

SEQ ID NO: 143 - DNA, 42 bp, synthetic construct
  misc_feature 1..42: note = source = /note="Description of Artificial Sequence: Synthetic oligonucleotide"
  source 1..42: mol_type = other DNA
tgggtccgccaggctccagggaaggggctggagtgggtcagt

SEQ ID NO: 144 - protein, 32 aa, synthetic construct
  REGION 1..32: note = source = /note="Description of Artificial Sequence: Synthetic polypeptide"
RFTISRDDSKNTAYLQMNSLKTEDTAVYYCAR

SEQ ID NO: 145 - DNA, 96 bp, synthetic construct
  misc_feature 1..96: note = source = /note="Description of Artificial Sequence: Synthetic oligonucleotide"
  source 1..96: mol_type = other DNA
agattcaccatctccagagatgattcaaagaacacggcgtatctgcaaatgaacagcctgaaaaccgaggacacggccgtgtattactgtgcaagg

SEQ ID NO: 146 - protein, 32 aa, synthetic construct
  REGION 1..32: note = source = /note="Description of Artificial Sequence: Synthetic polypeptide"
RVTITADKSTSTAYMELSSLRSEDTAVYYCAR

SEQ ID NO: 147 - DNA, 96 bp, synthetic construct
  misc_feature 1..96: note = source = /note="Description of Artificial Sequence: Synthetic oligonucleotide"
  source 1..96: mol_type = other DNA
agagtcacgattaccgcggacaaatccacgagcacagcctacatggagctgagcagcctgagatctgaggacacggccgtgtattactgtgcaagg

SEQ ID NO: 148 - protein, 32 aa, synthetic construct
  REGION 1..32: note = source = /note="Description of Artificial Sequence: Synthetic polypeptide"
RVTISVDTSKNQFSLKLSSVTAADTAVYYCAR

SEQ ID NO: 149 - DNA, 96 bp, synthetic construct
  misc_feature 1..96: note = source = /note="Description of Artificial Sequence: Synthetic oligonucleotide"
  source 1..96: mol_type = other DNA
agagtcaccatatcagtagacacgtccaagaaccagttctccctgaagctgagctctgtgaccgccgcggacacggctgtgtattactgtgcaagg

SEQ ID NO: 150 - protein, 32 aa, synthetic construct
  REGION 1..32: note = source = /note="Description of Artificial Sequence: Synthetic polypeptide"
RLTISKDTSKNQVVLTMTNMDPVDTATYYCAR

SEQ ID NO: 151 - DNA, 96 bp, synthetic construct
  misc_feature 1..96: note = source = /note="Description of Artificial Sequence: Synthetic oligonucleotide"
  source 1..96: mol_type = other DNA
agactcaccatctccaaggacacctccaaaaaccaggtggtccttacaatgaccaacatggaccctgtggacacagccacgtattactgtgcaagg

SEQ ID NO: 152 - protein, 32 aa, synthetic construct
  REGION 1..32: note = source = /note="Description of Artificial Sequence: Synthetic polypeptide"
RFTISRDNSKNTLYLQMNSLRAEDTAVYYCAR

SEQ ID NO: 153 - DNA, 96 bp, synthetic construct
  misc_feature 1..96: note = source = /note="Description of Artificial Sequence: Synthetic oligonucleotide"
  source 1..96: mol_type = other DNA
agattcaccatctccagagacaattccaagaacacgctgtatcttcaaatgaacagcctgagagccgaggacacggccgtgtattactgtgcaagg

SEQ ID NO: 154 - protein, 11 aa, synthetic construct
  REGION 1..11: note = source = /note="Description of Artificial Sequence: Synthetic peptide"
WGQGTTVTVSS

SEQ ID NO: 155 - DNA, 33 bp, synthetic construct
  misc_feature 1..33: note = source = /note="Description of Artificial Sequence: Synthetic oligonucleotide"
  source 1..33: mol_type = other DNA
tggggccagggcaccaccgtgaccgtgtcctcc

SEQ ID NO: 156 - protein, 23 aa, synthetic construct
  REGION 1..23: note = source = /note="Description of Artificial Sequence: Synthetic peptide"
EIVLTQSPDFQSVTPKEKVTITC

SEQ ID NO: 157 - DNA, 69 bp, synthetic construct
  misc_feature 1..69: note = source = /note="Description of Artificial Sequence: Synthetic oligonucleotide"
  source 1..69: mol_type = other DNA
gaaattgtgctgactcagtctccagactttcagtctgtgactccaaaggagaaagtcaccatcacctgc

SEQ ID NO: 158 - protein, 23 aa, synthetic construct
  REGION 1..23: note = source = /note="Description of Artificial Sequence: Synthetic peptide"
DVVMTQSPLSLPVTLGQPASISC

SEQ ID NO: 159 - DNA, 69 bp, synthetic construct
  misc_feature 1..69: note = source = /note="Description of Artificial Sequence: Synthetic oligonucleotide"
  source 1..69: mol_type = other DNA
gatgttgtgatgactcagtctccactctccctgcccgtcacccttggacagccggcctccatctcctgc

SEQ ID NO: 160 - protein, 23 aa, synthetic construct
  REGION 1..23: note = source = /note="Description of Artificial Sequence: Synthetic peptide"
DIVMTQTPLSLPVTPGEPASISC

SEQ ID NO: 161 - DNA, 69 bp, synthetic construct
  misc_feature 1..69: note = source = /note="Description of Artificial Sequence: Synthetic oligonucleotide"
  source 1..69: mol_type = other DNA
gatattgtgatgacccagactccactctccctgcccgtcacccctggagagccggcctccatctcctgc

SEQ ID NO: 162 - protein, 23 aa, synthetic construct
  REGION 1..23: note = source = /note="Description of Artificial Sequence: Synthetic peptide"
DIQMTQSPSSLSASVGDRVTITC

SEQ ID NO: 163 - DNA, 69 bp, synthetic construct
  misc_feature 1..69: note = source = /note="Description of Artificial Sequence: Synthetic oligonucleotide"
  source 1..69: mol_type = other DNA
gacatccagatgacccagtctccatcctccctgtctgcatctgtaggagacagagtcaccatcacttgc

SEQ ID NO: 164 - protein, 23 aa, synthetic construct
  REGION 1..23: note = source = /note="Description of Artificial Sequence: Synthetic peptide"
EIVLTQSPATLSLSPGERATLSC

SEQ ID NO: 165 - DNA, 69 bp, synthetic construct
  misc_feature 1..69: note = source = /note="Description of Artificial Sequence: Synthetic oligonucleotide"
  source 1..69: mol_type = other DNA
gaaattgtgttgacacagtctccagccaccctgtctttgtctccaggggaaagagccaccctctcctgc

SEQ ID NO: 166 - protein, 23 aa, synthetic construct
  REGION 1..23: note = source = /note="Description of Artificial Sequence: Synthetic peptide"
AIQLTQSPSSLSASVGDRVTITC

SEQ ID NO: 167 - DNA, 69 bp, synthetic construct
  misc_feature 1..69: note = source = /note="Description of Artificial Sequence: Synthetic oligonucleotide"
  source 1..69: mol_type = other DNA
gccatccagttgacccagtctccatcctccctgtctgcatctgtaggagacagagtcaccatcacttgc

SEQ ID NO: 168 - protein, 15 aa, synthetic construct
  REGION 1..15: note = source = /note="Description of Artificial Sequence: Synthetic peptide"
WYQQKPGQAPRLLIY

SEQ ID NO: 169 - DNA, 45 bp, synthetic construct
  misc_feature 1..45: note = source = /note="Description of Artificial Sequence: Synthetic oligonucleotide"
  source 1..45: mol_type = other DNA
tggtaccagcagaaacctggccaggctcccaggctcctcatctat

SEQ ID NO: 170 - protein, 15 aa, synthetic construct
  REGION 1..15: note = source = /note="Description of Artificial Sequence: Synthetic peptide"
WYLQKPGQSPQLLIY

SEQ ID NO: 171 - DNA, 45 bp, synthetic construct
  misc_feature 1..45: note = source = /note="Description of Artificial Sequence: Synthetic oligonucleotide"
  source 1..45: mol_type = other DNA
tggtacctgcagaagccagggcagtctccacagctcctgatctat

SEQ ID NO: 172 - protein, 32 aa, synthetic construct
  REGION 1..32: note = source = /note="Description of Artificial Sequence: Synthetic polypeptide"
GVPSRFSGSGSGTEFTLTISSLQPDDFATYYC

SEQ ID NO: 173 - DNA, 96 bp, synthetic construct
  misc_feature 1..96: note = source = /note="Description of Artificial Sequence: Synthetic oligonucleotide"
  source 1..96: mol_type = other DNA
ggggtcccatcaaggttcagcggcagtggatctgggacagaattcactctcaccatcagcagcctgcagcctgatgattttgcaacttattactgt

SEQ ID NO: 174 - protein, 32 aa, synthetic construct
  REGION 1..32: note = source = /note="Description of Artificial Sequence: Synthetic polypeptide"
GVPSRFSGSGSGTDFTFTISSLQPEDIATYYC

SEQ ID NO: 175 - DNA, 96 bp, synthetic construct
  misc_feature 1..96: note = source = /note="Description of Artificial Sequence: Synthetic oligonucleotide"
  source 1..96: mol_type = other DNA
ggggtcccatcaaggttcagtggaagtggatctgggacagattttactttcaccatcagcagcctgcagcctgaagatattgcaacatattactgt

SEQ ID NO: 176 - protein, 32 aa, synthetic construct
  REGION 1..32: note = source = /note="Description of Artificial Sequence: Synthetic polypeptide"
GIPARFSGSGSGTEFTLTISSLQSEDFAVYYC

SEQ ID NO: 177 - DNA, 96 bp, synthetic construct
  misc_feature 1..96: note = source = /note="Description of Artificial Sequence: Synthetic oligonucleotide"
  source 1..96: mol_type = other DNA
gggatcccagccaggttcagtggcagtgggtctgggacagagttcactctcaccatcagcagcctgcagtctgaagattttgcagtttattactgt

SEQ ID NO: 178 - protein, 32 aa, synthetic construct
  REGION 1..32: note = source = /note="Description of Artificial Sequence: Synthetic polypeptide"
GVPSRFSGSGSGTDFTLTISSLQPEDFATYYC

SEQ ID NO: 179 - DNA, 96 bp, synthetic construct
  misc_feature 1..96: note = source = /note="Description of Artificial Sequence: Synthetic oligonucleotide"
  source 1..96: mol_type = other DNA
ggggtcccatcaaggttcagcggcagtggatctgggacagatttcactctcaccatcagcagcctgcagcctgaagattttgcaacttattactgt

SEQ ID NO: 180 - protein, 32 aa, synthetic construct
  REGION 1..32: note = source = /note="Description of Artificial Sequence: Synthetic polypeptide"
GVPDRFSGSGSGTDFTLKISRVEAEDVGVYYC

SEQ ID NO: 181 - DNA, 96 bp, synthetic construct
  misc_feature 1..96: note = source = /note="Description of Artificial Sequence: Synthetic oligonucleotide"
  source 1..96: mol_type = other DNA
ggggtcccagacaggttcagtggcagtgggtcaggcactgatttcacactgaaaatcagcagggtggaggctgaggatgttggagtttattactgt

SEQ ID NO: 182 - protein, 32 aa, synthetic construct
  REGION 1..32: note = source = /note="Description of Artificial Sequence: Synthetic polypeptide"
GIPPRFSGSGYGTDFTLTINNIESEDAAYYFC

SEQ ID NO: 183 - DNA, 96 bp, synthetic construct
  misc_feature 1..96: note = source = /note="Description of Artificial Sequence: Synthetic oligonucleotide"
  source 1..96: mol_type = other DNA
gggatcccacctcgattcagtggcagcgggtatggaacagattttaccctcacaattaataacatagaatctgaggatgctgcatattacttctgt

SEQ ID NO: 184 - protein, 32 aa, synthetic construct
  REGION 1..32: note = source = /note="Description of Artificial Sequence: Synthetic polypeptide"
GVPSRFSGSGSGTDFTFTISSLEAEDAATYYC

SEQ ID NO: 185 - DNA, 96 bp, synthetic construct
  misc_feature 1..96: note = source = /note="Description of Artificial Sequence: Synthetic oligonucleotide"
  source 1..96: mol_type = other DNA
ggggtcccctcgaggttcagtggcagtggatctgggacagatttcacctttaccatcagtagcctggaagctgaagatgctgcaacatattactgt

SEQ ID NO: 186 - protein, 10 aa, synthetic construct
  REGION 1..10: note = source = /note="Description of Artificial Sequence: Synthetic peptide"
FGQGTKVEIK

SEQ ID NO: 187 - DNA, 30 bp, synthetic construct
  misc_feature 1..30: note = source = /note="Description of Artificial Sequence: Synthetic oligonucleotide"
  source 1..30: mol_type = other DNA
ttcggccaagggaccaaggtggaaatcaaa

SEQ ID NO: 188 - protein, 327 aa, synthetic construct
  REGION 1..327: note = source = /note="Description of Artificial Sequence: Synthetic polypeptide"
ASTKGPSVFPLAPCSRSTSESTAALGCLVKDYFPEPVTVSWNSGALTSGVHTFPAVLQSSGLYSLSSVVTVPSSSLGTKTYTCNVDHKPSNTKVDKRVESKYGPPCPPCPAPEFLGGPSVFLFPPKPKDTLMISRTPEVTCVVVDVSQEDPEVQFNWYVDGVEVHNAKTKPREEQFNSTYRVVSVLTVLHQDWLNGKEYKCKVSNKGLPSSIEKTISKAKGQPREPQVYTLPPSQEEMTKNQVSLTCLVKGFYPSDIAVEWESNGQPENNYKTTPPVLDSDGSFFLYSRLTVDKSRWQEGNVFSCSVMHEALHNHYTQKSLSLSLGK

SEQ ID NO: 189 - protein, 107 aa, synthetic construct [sequence omitted]

SEQ ID NO: 190 - protein, 326 aa, synthetic construct
  REGION 1..326: note = source = /note="Description of Artificial Sequence: Synthetic polypeptide"
ASTKGPSVFPLAPCSRSTSESTAALGCLVKDYFPEPVTVSWNSGALTSGVHTFPAVLQSSGLYSLSSVVTVPSSSLGTKTYTCNVDHKPSNTKVDKRVESKYGPPCPPCPAPEFLGGPSVFLFPPKPKDTLMISRTPEVTCVVVDVSQEDPEVQFNWYVDGVEVHNAKTKPREEQFNSTYRVVSVLTVLHQDWLNGKEYKCKVSNKGLPSSIEKTISKAKGQPREPQVYTLPPSQEEMTKNQVSLTCLVKGFYPSDIAVEWESNGQPENNYKTTPPVLDSDGSFFLYSRLTVDKSRWQEGNVFSCSVMHEALHNHYTQKSLSLSLG

SEQ ID NO: 191 - protein, 330 aa, synthetic construct
  REGION 1..330: note = source = /note="Description of Artificial Sequence: Synthetic polypeptide"
ASTKGPSVFPLAPSSKSTSGGTAALGCLVKDYFPEPVTVSWNSGALTSGVHTFPAVLQSSGLYSLSSVVTVPSSSLGTQTYICNVNHKPSNTKVDKRVEPKSCDKTHTCPPCPAPELLGGPSVFLFPPKPKDTLMISRTPEVTCVVVDVSHEDPEVKFNWYVDGVEVHNAKTKPREEQYNSTYRVVSVLTVLHQDWLNGKEYKCKVSNKALPAPIEKTISKAKGQPREPQVYTLPPSREEMTKNQVSLTCLVKGFYPSDIAVEWESNGQPENNYKTTPPVLDSDGSFFLYSKLTVDKSRWQQGNVFSCSVMHEALHNHYTQKSLSLSPGK

SEQ ID NO: 192 - protein, 330 aa, synthetic construct
  REGION 1..330: note = source = /note="Description of Artificial Sequence: Synthetic polypeptide"
ASTKGPSVFPLAPSSKSTSGGTAALGCLVKDYFPEPVTVSWNSGALTSGVHTFPAVLQSSGLYSLSSVVTVPSSSLGTQTYICNVNHKPSNTKVDKRVEPKSCDKTHTCPPCPAPELLGGPSVFLFPPKPKDTLMISRTPEVTCVVVDVSHEDPEVKFNWYVDGVEVHNAKTKPREEQYASTYRVVSVLTVLHQDWLNGKEYKCKVSNKALPAPIEKTISKAKGQPREPQVYTLPPSREEMTKNQVSLTCLVKGFYPSDIAVEWESNGQPENNYKTTPPVLDSDGSFFLYSKLTVDKSRWQQGNVFSCSVMHEALHNHYTQKSLSLSPGK

SEQ ID NO: 193 - protein, 330 aa, synthetic construct
  REGION 1..330: note = source = /note="Description of Artificial Sequence: Synthetic polypeptide"
ASTKGPSVFPLAPSSKSTSGGTAALGCLVKDYFPEPVTVSWNSGALTSGVHTFPAVLQSSGLYSLSSVVTVPSSSLGTQTYICNVNHKPSNTKVDKRVEPKSCDKTHTCPPCPAPELLGGPSVFLFPPKPKDTLMISRTPEVTCVVVAVSHEDPEVKFNWYVDGVEVHNAKTKPREEQYNSTYRVVSVLTVLHQDWLNGKEYKCKVSNKALAAPIEKTISKAKGQPREPQVYTLPPSREEMTKNQVSLTCLVKGFYPSDIAVEWESNGQPENNYKTTPPVLDSDGSFFLYSKLTVDKSRWQQGNVFSCSVMHEALHNHYTQKSLSLSPGK

SEQ ID NO: 194 - protein, 330 aa, synthetic construct
  REGION 1..330: note = source = /note="Description of Artificial Sequence: Synthetic polypeptide"
ASTKGPSVFPLAPSSKSTSGGTAALGCLVKDYFPEPVTVSWNSGALTSGVHTFPAVLQSSGLYSLSSVVTVPSSSLGTQTYICNVNHKPSNTKVDKRVEPKSCDKTHTCPPCPAPEAAGGPSVFLFPPKPKDTLMISRTPEVTCVVVDVSHEDPEVKFNWYVDGVEVHNAKTKPREEQYNSTYRVVSVLTVLHQDWLNGKEYKCKVSNKALPAPIEKTISKAKGQPREPQVYTLPPSREEMTKNQVSLTCLVKGFYPSDIAVEWESNGQPENNYKTTPPVLDSDGSFFLYSKLTVDKSRWQQGNVFSCSVMHEALHNHYTQKSLSLSPGK

SEQ ID NO: 195 - protein, 10 aa, synthetic construct
  REGION 1..10: note = source = /note="Description of Artificial Sequence: Synthetic peptide"
GYTFTSYWMY

SEQ ID NO: 196 - DNA, 360 bp, synthetic construct
  misc_feature 1..360: note = source = /note="Description of Artificial Sequence: Synthetic polynucleotide"
  source 1..360: mol_type = other DNA
gaagtgcagctggtgcagtctggcgccgaagtgaagaaacccggcgctaccgtgaagatctcctgcaaggtgtccggctacaccttcaccagctactggatgtactgggtgcgacaggctaccggccagggcctggaatggatgggcagaatcgaccccaactccggctccaccaagtacaacgagaagttcaagaaccgcgtgaccatcaccgccgacaagtccacctccaccgcctacatggaactgtcctccctgcggagcgaggacaccgccgtgtactactgcgccagagactaccggaagggcctgtacgccatggactattggggccagggcaccaccgtgaccgtgtcctct

SEQ ID NO: 197 - protein, 446 aa, synthetic construct; identical to SEQ ID NO: 96
  REGION 1..446: note = source = /note="Description of Artificial Sequence: Synthetic polypeptide"

SEQ ID NO: 198 - DNA, 1348 bp, synthetic construct
  misc_feature 1..1348: note = source = /note="Description of Artificial Sequence: Synthetic polynucleotide"
  source 1..1348: mol_type = other DNA
gaagtgcagctggtgcagtctggcgccgaagtgaagaaacccggcgctaccgtgaagatctcctgcaaggtgtccggctacaccttcaccagctactggatgtactgggtgcgacaggctaccggccagggcctggaatggatgggcagaatcgaccccaactccggctccaccaagtacaacgagaagttcaagaaccgcgtgaccatcaccgccgacaagtccacctccaccgcctacatggaactgtcctccctgcggagcgaggacaccgccgtgtactactgcgccagagactaccggaagggcctgtacgccatggactattggggccagggcaccaccgtgaccgtgtcctctgcttccaccaagggcccaagcgtgttccccctggccccctgctccagaagcaccagcgagagcacagccgccctgggctgcctggtgaaggactacttccccgagcccgtgaccgtgtcctggaacagcggagccctgaccagcggcgtgcacaccttccccgccgtgctgcagagcagcggcctgtacagcctgagcagcgtggtgaccgtgcccagcagcagcctgggcaccaagacctacacctgtaacgtggaccacaagcccagcaacaccaaggtggacaagagggtggagagcaagtacggcccaccctgccccccctgcccagcccccgagttcctgggcggacccagcgtgttcctgttcccccccaagcccaaggacaccctgatgatcagcagaacccccgaggtgacctgtgtggtggtggacgtgtcccaggaggaccccgaggtccagttcaactggtacgtggacggcgtggaggtgcacaacgccaagaccaagcccagagaggagcagtttaacagcacctaccgggtggtgtccgtgctgaccgtgctgcaccaggactggctgaacggcaaagagtacaagtgtaaggtctccaacaagggcctgccaagcagcatcgaaaagaccatcagcaaggccaagggccagcctagagagccccaggtctacaccctgccacccagccaagaggagatgaccaagaaccaggtgtccctgacctgtctggtgaagggcttctacccaagcgacatcgccgtggagtgggagagcaacggccagcccgagaacaactacaagaccacccccccagtgctggacagcgacggcagcttcttcctgtacagcaggctgaccgtggacaagtccagatggcaggagggcaacgtctttagctgctccgtgatgcacgaggccctgcacaaccactacacccagaagagcctgagcctgtccctgggctgatgaattc

SEQ ID NO: 199 - DNA, 321 bp, synthetic construct
  misc_feature 1..321: note = source = /note="Description of Artificial Sequence: Synthetic polynucleotide"
  source 1..321: mol_type = other DNA
gagatcgtgctgacccagtcccccgacttccagtccgtgacccccaaagaaaaagtgaccatcacatgcaaggcctcccaggacgtgggcaccgccgtggcttggtatctgcagaagcctggccagtcccctcagctgctgatctactgggcctctaccagacacaccggcgtgcccgacagattctccggctctggctctggcaccgacttcaccctgaagatctcccgggtggaagccgaggatgtgggcgtgtactactgccagcagtacaactcctaccccctgaccttcggccagggcaccaaggtggaaatcaag

SEQ ID NO: 200 - DNA, 652 bp, synthetic construct
  misc_feature 1..652: note = source = /note="Description of Artificial Sequence: Synthetic polynucleotide"
  source 1..652: mol_type = other DNA
gagatcgtgctgacccagtcccccgacttccagtccgtgacccccaaagaaaaagtgaccatcacatgcaaggcctcccaggacgtgggcaccgccgtggcttggtatctgcagaagcctggccagtcccctcagctgctgatctactgggcctctaccagacacaccggcgtgcccgacagattctccggctctggctctggcaccgacttcaccctgaagatctcccgggtggaagccgaggatgtgggcgtgtactactgccagcagtacaactcctaccccctgaccttcggccagggcaccaaggtggaaatcaagcgtacggtggccgctcccagcgtgttcatcttccccccaagcgacgagcagctgaagagcggcaccgccagcgtggtgtgtctgctgaacaacttctaccccagggaggccaaggtgcagtggaaggtggacaacgccctgcagagcggcaacagccaggagagcgtcaccgagcaggacagcaaggactccacctacagcctgagcagcaccctgaccctgagcaaggccgactacgagaagcacaaggtgtacgcctgtgaggtgacccaccagggcctgtccagccccgtgaccaagagcttcaacaggggcgagtgctgatgaattc

SEQ ID NO: 201 - DNA, 360 bp, synthetic construct
  misc_feature 1..360: note = source = /note="Description of Artificial Sequence: Synthetic polynucleotide"
  source 1..360: mol_type = other DNA
gaagtgcagctggtgcagtctggcgccgaagtgaagaagcctggcgagtccctgcggatctcctgcaagggctccggctacaccttcaccagctactggatgtactggatccggcagccccctggcaagggcctggaatggatcggcagaatcgaccccaactccggctccaccaagtacaacgagaagttcaagaaccgcgtgaccatcaccgccgacaagtccacctccaccgcctacatggaactgtcctccctgagatccgaggacaccgccgtgtactactgcgccagagactaccggaagggcctgtacgccatggactattggggccagggcaccaccgtgaccgtgtcctct

SEQ ID NO: 202 - DNA, 1348 bp, synthetic construct
  misc_feature 1..1348: note = source = /note="Description of Artificial Sequence: Synthetic polynucleotide"
  source 1..1348: mol_type = other DNA
gaagtgcagctggtgcagtctggcgccgaagtgaagaagcctggcgagtccctgcggatctcctgcaagggctccggctacaccttcaccagctactggatgtactggatccggcagccccctggcaagggcctggaatggatcggcagaatcgaccccaactccggctccaccaagtacaacgagaagttcaagaaccgcgtgaccatcaccgccgacaagtccacctccaccgcctacatggaactgtcctccctgagatccgaggacaccgccgtgtactactgcgccagagactaccggaagggcctgtacgccatggactattggggccagggcaccaccgtgaccgtgtcctctgcttctaccaagggcccaagcgtgttccccctggccccctgctccagaagcaccagcgagagcacagccgccctgggctgcctggtgaaggactacttccccgagcccgtgaccgtgtcctggaacagcggagccctgaccagcggcgtgcacaccttccccgccgtgctgcagagcagcggcctgtacagcctgagcagcgtggtgaccgtgcccagcagcagcctgggcaccaagacctacacctgtaacgtggaccacaagcccagcaacaccaaggtggacaagagggtggagagcaagtacggcccaccctgccccccctgcccagcccccgagttcctgggcggacccagcgtgttcctgttcccccccaagcccaaggacaccctgatgatcagcagaacccccgaggtgacctgtgtggtggtggacgtgtcccaggaggaccccgaggtccagttcaactggtacgtggacggcgtggaggtgcacaacgccaagaccaagcccagagaggagcagtttaacagcacctaccgggtggtgtccgtgctgaccgtgctgcaccaggactggctgaacggcaaagagtacaagtgtaaggtctccaacaagggcctgccaagcagcatcgaaaagaccatcagcaaggccaagggccagcctagagagccccaggtctacaccctgccacccagccaagaggagatgaccaagaaccaggtgtccctgacctgtctggtgaagggcttctacccaagcgacatcgccgtggagtgggagagcaacggccagcccgagaacaactacaagaccacccccccagtgctggacagcgacggcagcttcttcctgtacagcaggctgaccgtggacaagtccagatggcaggagggcaacgtctttagctgctccgtgatgcacgaggccctgcacaaccactacacccagaagagcctgagcctgtccctgggctgatgaattc

SEQ ID NO: 203 - DNA, 321 bp, synthetic construct
  misc_feature 1..321: note = source = /note="Description of Artificial Sequence: Synthetic polynucleotide"
  source 1..321: mol_type = other DNA
gagatcgtgctgacccagtcccccgacttccagtccgtgacccccaaagaaaaagtgaccatcacatgcaaggcctcccaggacgtgggcaccgccgtggcttggtatctgcagaagcctggccagtcccctcagctgctgatctactgggcctctaccagacacaccggcgtgccctccagattctccggctctggctctggcaccgactttaccttcaccatctccagcctgcagcccgaggatatcgccacctactactgccagcagtacaactcctaccccctgaccttcggccagggcaccaaggtggaaatcaag

SEQ ID NO: 204 - DNA, 652 bp, synthetic construct
  misc_feature 1..652: note = source = /note="Description of Artificial Sequence: Synthetic polynucleotide"
  source 1..652: mol_type = other DNA
gagatcgtgctgacccagtcccccgacttccagtccgtgacccccaaagaaaaagtgaccatcacatgcaaggcctcccaggacgtgggcaccgccgtggcttggtatctgcagaagcctggccagtcccctcagctgctgatctactgggcctctaccagacacaccggcgtgccctccagattctccggctctggctctggcaccgactttaccttcaccatctccagcctgcagcccgaggatatcgccacctactactgccagcagtacaactcctaccccctgaccttcggccagggcaccaaggtggaaatcaagcgtacggtggccgctcccagcgtgttcatcttccccccaagcgacgagcagctgaagagcggcaccgccagcgtggtgtgtctgctgaacaacttctaccccagggaggccaaggtgcagtggaaggtggacaacgccctgcagagcggcaacagccaggagagcgtcaccgagcaggacagcaaggactccacctacagcctgagcagcaccctgaccctgagcaaggccgactacgagaagcacaaggtgtacgcctgtgaggtgacccaccagggcctgtccagccccgtgaccaagagcttcaacaggggcgagtgctgatgaattc

SEQ ID NO: 205 - DNA, 51 bp, synthetic construct
  misc_feature 1..51: note = source = /note="Description of Artificial Sequence: Synthetic oligonucleotide"
  source 1..51: mol_type = other DNA
agaatcgaccccaactccggctccaccaagtacaacgagaagttcaagaac

SEQ ID NO: 206 - DNA, 33 bp, synthetic construct
  misc_feature 1..33: note = source = /note="Description of Artificial Sequence: Synthetic oligonucleotide"
  source 1..33: mol_type = other DNA
gactaccggaagggcctgtacgccatggactat

SEQ ID NO: 207 - DNA, 21 bp, synthetic construct
  misc_feature 1..21: note = source = /note="Description of Artificial Sequence: Synthetic oligonucleotide"
  source 1..21: mol_type = other DNA
ggctacaccttcaccagctac

SEQ ID NO: 208 - DNA, 18 bp, synthetic construct
  misc_feature 1..18: note = source = /note="Description of Artificial Sequence: Synthetic oligonucleotide"
  source 1..18: mol_type = other DNA
gaccccaactccggctcc

SEQ ID NO: 209 - DNA, 33 bp, synthetic construct
  misc_feature 1..33: note = source = /note="Description of Artificial Sequence: Synthetic oligonucleotide"
  source 1..33: mol_type = other DNA
aaggcctcccaggacgtgggcaccgccgtggct

SEQ ID NO: 210 - DNA, 21 bp, synthetic construct
  misc_feature 1..21: note = source = /note="Description of Artificial Sequence: Synthetic oligonucleotide"
  source 1..21: mol_type = other DNA
tgggcctctaccagacacacc

SEQ ID NO: 211 - DNA, 27 bp, synthetic construct
  misc_feature 1..27: note = source = /note="Description of Artificial Sequence: Synthetic oligonucleotide"
  source 1..27: mol_type = other DNA
cagcagtacaactcctaccccctgacc

SEQ ID NO: 212 - DNA, 21 bp, synthetic construct
  misc_feature 1..21: note = source = /note="Description of Artificial Sequence: Synthetic oligonucleotide"
  source 1..21: mol_type = other DNA
tcccaggacgtgggcaccgcc

SEQ ID NO: 213 - skipped

SEQ ID NO: 214 - DNA, 18 bp, synthetic construct
  misc_feature 1..18: note = source = /note="Description of Artificial Sequence: Synthetic oligonucleotide"
  source 1..18: mol_type = other DNA
tacaactcctaccccctg

SEQ ID NO: 215 - DNA, 75 bp, synthetic construct
  misc_feature 1..75: note = source = /note="Description of Artificial Sequence: Synthetic oligonucleotide"
  source 1..75: mol_type = other DNA
gaagtgcagctggtgcagtcaggcgccgaagtgaagaagcccggcgagtcactgagaattagctgtaaaggttca

SEQ ID NO: 216 - DNA, 75 bp, synthetic construct
  misc_feature 1..75: note = source = /note="Description of Artificial Sequence: Synthetic oligonucleotide"
  source 1..75: mol_type = other DNA
gaagtgcagctggtgcagtctggcgccgaagtgaagaagcctggcgagtccctgcggatctcctgcaagggctcc

SEQ ID NO: 217 - DNA, 75 bp, synthetic construct
  misc_feature 1..75: note = source = /note="Description of Artificial Sequence: Synthetic oligonucleotide"
  source 1..75: mol_type = other DNA
gaagtgcagctggtgcagtctggcgccgaagtgaagaaacccggcgctaccgtgaagatctcctgcaaggtgtcc

SEQ ID NO: 218 - DNA, 75 bp, synthetic construct
  misc_feature 1..75: note = source = /note="Description of Artificial Sequence: Synthetic oligonucleotide"
  source 1..75: mol_type = other DNA
gaagtgcagctggtgcagtcaggcgccgaagtgaagaaacccggcgctaccgtgaagattagctgtaaagtctca

SEQ ID NO: 219 - DNA, 42 bp, synthetic construct
  misc_feature 1..42: note = source = /note="Description of Artificial Sequence: Synthetic oligonucleotide"
  source 1..42: mol_type = other DNA
tgggtgcgacaggctaccggccagggcctggaatggatgggc

SEQ ID NO: 220 - DNA, 42 bp, synthetic construct
  misc_feature 1..42: note = source = /note="Description of Artificial Sequence: Synthetic oligonucleotide"
  source 1..42: mol_type = other DNA
tgggtccgacaggctaccggtcaaggcctggagtggatgggt

SEQ ID NO: 221 - DNA, 42 bp, synthetic construct
  misc_feature 1..42: note = source = /note="Description of Artificial Sequence: Synthetic oligonucleotide"
  source 1..42: mol_type = other DNA
tgggtccgacaggccccagggcaaggcctggagtggatgggt

SEQ ID NO: 222 - DNA, 42 bp, synthetic construct
  misc_feature 1..42: note = source = /note="Description of Artificial Sequence: Synthetic oligonucleotide"
  source 1..42: mol_type = other DNA
tggatccggcagccccctggcaagggcctggaatggatcggc

SEQ ID NO: 223 - DNA, 42 bp, synthetic construct
  misc_feature 1..42: note = source = /note="Description of Artificial Sequence: Synthetic oligonucleotide"
  source 1..42: mol_type = other DNA
tgggtccgacaggctagagggcaaagactggagtggatcggt

SEQ ID NO: 224 - DNA, 96 bp, synthetic construct
  misc_feature 1..96: note = source = /note="Description of Artificial Sequence: Synthetic oligonucleotide"
  source 1..96: mol_type = other DNA
cgcgtgaccatcaccgccgacaagtccacctccaccgcctacatggaactgtcctccctgcggagcgaggacaccgccgtgtactactgcgccaga

SEQ ID NO: 225 - DNA, 96 bp, synthetic construct
  misc_feature 1..96: note = source = /note="Description of Artificial Sequence: Synthetic oligonucleotide"
  source 1..96: mol_type = other DNA
cgcgtgaccatcaccgccgacaagtccacctccaccgcctacatggaactgtcctccctgagatccgaggacaccgccgtgtactactgcgccaga

SEQ ID NO: 226 - DNA, 96 bp, synthetic construct
  misc_feature 1..96: note = source = /note="Description of Artificial Sequence: Synthetic oligonucleotide"
  source 1..96: mol_type = other DNA
agagtgactatcaccgccgataagtctactagcaccgcctatatggaactgtctagcctgagatcagaggacaccgccgtctactactgcgctaga

SEQ ID NO: 227 - DNA, 96 bp, synthetic construct
  misc_feature 1..96: note = source = /note="Description of Artificial Sequence: Synthetic oligonucleotide"
  source 1..96: mol_type = other DNA
agagtgactattagcgtggacacctctaagaatcagtttagcctgaagctgtctagcgtgaccgccgctgacaccgccgtctactactgcgctaga

SEQ ID NO: 228 - DNA, 96 bp, synthetic construct
  misc_feature 1..96: note = source = /note="Description of Artificial Sequence: Synthetic oligonucleotide"
  source 1..96: mol_type = other DNA
aggttcactattagtagggataactctaagaacaccctgtacctgcagatgaatagcctgagagccgaggacaccgccgtctactactgcgctaga

SEQ ID NO: 229 - DNA, 33 bp, synthetic construct
  misc_feature 1..33: note = source = /note="Description of Artificial Sequence: Synthetic oligonucleotide"
  source 1..33: mol_type = other DNA
tggggccagggcaccaccgtgaccgtgtcctct

SEQ ID NO: 230 - DNA, 33 bp, synthetic construct
  misc_feature 1..33: note = source = /note="Description of Artificial Sequence: Synthetic oligonucleotide"
  source 1..33: mol_type = other DNA
tggggtcaaggcactaccgtgaccgtgtcttca

SEQ ID NO: 231 - DNA, 69 bp, synthetic construct
  misc_feature 1..69: note = source = /note="Description of Artificial Sequence: Synthetic oligonucleotide"
  source 1..69: mol_type = other DNA
gagatcgtgctgacccagtcccccgacttccagtccgtgacccccaaagaaaaagtgaccatcacatgc

SEQ ID NO: 232 - DNA, 69 bp, synthetic construct
  misc_feature 1..69: note = source = /note="Description of Artificial Sequence: Synthetic oligonucleotide"
  source 1..69: mol_type = other DNA
gagatcgtcctgactcagtcacccgactttcagtcagtgacccctaaagagaaagtcactatcacctgt

SEQ ID NO: 233 - DNA, 69 bp, synthetic construct
  misc_feature 1..69: note = source = /note="Description of Artificial Sequence: Synthetic oligonucleotide"
  source 1..69: mol_type = other DNA
gacgtcgtgatgactcagtcacccctgagcctgcccgtgaccctggggcagcccgcctctattagctgt

SEQ ID NO: 234 - DNA, 69 bp, synthetic construct
  misc_feature 1..69: note = source = /note="Description of Artificial Sequence: Synthetic oligonucleotide"
  source 1..69: mol_type = other DNA
gctattcagctgactcagtcacctagtagcctgagcgctagtgtgggcgatagagtgactatcacctgt

SEQ ID NO: 235 - DNA, 45 bp, synthetic construct
  misc_feature 1..45: note = source = /note="Description of Artificial Sequence: Synthetic oligonucleotide"
  source 1..45: mol_type = other DNA
tggtatcagcagaagccagggcaagcccctagactgctgatctac

SEQ ID NO: 236 - DNA, 45 bp, synthetic construct
  misc_feature 1..45: note = source = /note="Description of Artificial Sequence: Synthetic oligonucleotide"
  source 1..45: mol_type = other DNA
tggtatctgcagaagcctggccagtcccctcagctgctgatctac

SEQ ID NO: 237 - DNA, 45 bp, synthetic construct
  misc_feature 1..45: note = source = /note="Description of Artificial Sequence: Synthetic oligonucleotide"
  source 1..45: mol_type = other DNA
tggtatctgcagaagcctggtcaatcacctcagctgctgatctac

SEQ ID NO: 238 - DNA, 96 bp, synthetic construct
  misc_feature 1..96: note = source = /note="Description of Artificial Sequence: Synthetic oligonucleotide"
  source 1..96: mol_type = other DNA
ggcgtgccctctaggtttagcggtagcggtagtggcaccgagttcaccctgactatctcttcactgcagcccgacgacttcgctacctactactgt

SEQ ID NO: 239 - DNA, 96 bp, synthetic construct
  misc_feature 1..96: note = source = /note="Description of Artificial Sequence: Synthetic oligonucleotide"
  source 1..96: mol_type = other DNA
ggcgtgccctctaggtttagcggtagcggtagtggcaccgacttcaccttcactatctcttcactgcagcccgaggatatcgctacctactactgt

SEQ ID NO: 240 - DNA, 96 bp, synthetic construct
  misc_feature 1..96: note = source = /note="Description of Artificial Sequence: Synthetic oligonucleotide"
  source 1..96: mol_type = other DNA
ggcgtgccctccagattctccggctctggctctggcaccgactttaccttcaccatctccagcctgcagcccgaggatatcgccacctactactgc

SEQ ID NO: 241 - DNA, 96 bp, synthetic construct
  misc_feature 1..96: note = source = /note="Description of Artificial Sequence: Synthetic oligonucleotide"
  source 1..96: mol_type = other DNA
ggcgtgcccgacagattctccggctctggctctggcaccgacttcaccctgaagatctcccgggtggaagccgaggatgtgggcgtgtactactgc

SEQ ID NO: 242 - DNA, 96 bp, synthetic construct
  misc_feature 1..96: note = source = /note="Description of Artificial Sequence: Synthetic oligonucleotide"
  source 1..96: mol_type = other DNA
ggcgtgccctctaggtttagcggtagcggtagtggcaccgacttcaccttcactatctcttcactggaagccgaggacgccgctacctactactgt

SEQ ID NO: 243 - DNA, 30 bp, synthetic construct
  misc_feature 1..30: note = source = /note="Description of Artificial Sequence: Synthetic oligonucleotide"
  source 1..30: mol_type = other DNA
ttcggccagggcaccaaggtggaaatcaag

SEQ ID NO: 244 - DNA, 30 bp, synthetic construct
  misc_feature 1..30: note = source = /note="Description of Artificial Sequence: Synthetic oligonucleotide"
  source 1..30: mol_type = other DNA
ttcggtcaaggcactaaggtcgagattaag

SEQ ID NO: 245 - DNA, 33 bp, synthetic construct
  misc_feature 1..33: note = source = /note="Description of Artificial Sequence: Synthetic oligonucleotide"
  source 1..33: mol_type = other DNA
aaggccagtcaggatgtgggtactgctgtagcc

SEQ ID NO: 246 - DNA, 21 bp, synthetic construct
  misc_feature 1..21: note = source = /note="Description of Artificial Sequence: Synthetic oligonucleotide"
  source 1..21: mol_type = other DNA
tgggcatccacccggcacact

SEQ ID NO: 247 - protein, 447 aa, synthetic construct
  REGION 1..447: note = source = /note="Description of Artificial Sequence: Synthetic polypeptide"
EVQLVQSGAEVKKPGATVKISCKVSGYTFTSYWMYWVRQARGQRLEWIGRIDPNSGSTKYNEKFKNRFTISRDNSKNTLYLQMNSLRAEDTAVYYCARDYRKGLYAMDYWGQGTTVTVSSASTKGPSVFPLAPCSRSTSESTAALGCLVKDYFPEPVTVSWNSGALTSGVHTFPAVLQSSGLYSLSSVVTVPSSSLGTKTYTCNVDHKPSNTKVDKRVESKYGPPCPPCPAPEFLGGPSVFLFPPKPKDTLMISRTPEVTCVVVDVSQEDPEVQFNWYVDGVEVHNAKTKPREEQFNSTYRVVSVLTVLHQDWLNGKEYKCKVSNKGLPSSIEKTISKAKGQPREPQVYTLPPSQEEMTKNQVSLTCLVKGFYPSDIAVEWESNGQPENNYKTTPPVLDSDGSFFLYSRLTVDKSRWQEGNVFSCSVMHEALHNHYTQKSLSLSLGK

SEQ ID NO: 248 - protein, 98 aa, synthetic construct
  REGION 1..98: note = source = /note="Description of Artificial Sequence: Synthetic polypeptide"
QVQLQQPGAELVKPGASVKLSCKASGYTFTSYWMHWVKQRPGRGLEWIGRIDPNSGGTKYNEKFKSKATLTVDKPSSTAYMQLSSLTSEDSAVYYCAR

SEQ ID NO: 249 - protein, 107 aa, synthetic construct
  REGION 1..107: note = source = /note="Description of Artificial Sequence: Synthetic polypeptide"
DIVMTQSHKFMSTSVGDRVSITCKASQDVGTAVAWYQQKPGQSPKLLIYWASTRHTGVPDRFTGSGSGTDFTLTISNVQSEDLADYFCQQYSSYPLTFGAGSKLELK

SEQ ID NO: 250 - protein, 113 aa, synthetic construct
  REGION 1..113: note = source = /note="Description of Artificial Sequence: Synthetic polypeptide"
EVQLQQSGAELVKPGASVKLSCKASGYTFTSYWMYWVKQGPGRGLEWIGRIDPNSGSTKYNEKFKNKATLTVDKSSSTAYMQLSSLTSEDSAVYYCARDYRKGLYAMDYWGQG

SEQ ID NO: 251 - protein, 113 aa, synthetic construct
  REGION 1..113: note = source = /note="Description of Artificial Sequence: Synthetic polypeptide"
QVQLVQSGAEVKKPGASVKVSCKASGYTFTSYWMYWVRQATGQGLEWMGRIDPNSGSTKYNEKFKNRFTISRDDSKNTAYLQMNSLKTEDTAVYYCARDYRKGLYAMDYWGQG

SEQ ID NO: 252 - protein, 113 aa, synthetic construct
  REGION 1..113: note = source = /note="Description of Artificial Sequence: Synthetic polypeptide"
EVQLVQSGAEVKKPGESLRISCKGSGYTFTSYWMYWIRQPPGKGLEWIGRIDPNSGSTKYNEKFKNRVTITADKSTSTAYMELSSLRSEDTAVYYCARDYRKGLYAMDYWGQG

SEQ ID NO: 253 - protein, 113 aa, synthetic construct
  REGION 1..113: note = source = /note="Description of Artificial Sequence: Synthetic polypeptide"
EVQLVQSGAEVKKPGATVKISCKVSGYTFTSYWMYWVRQATGQGLEWMGRIDPNSGSTKYNEKFKNRVTITADKSTSTAYMELSSLRSEDTAVYYCARDYRKGLYAMDYWGQG

SEQ ID NO: 254 - protein, 113 aa, synthetic construct
  REGION 1..113: note = source = /note="Description of Artificial Sequence: Synthetic polypeptide"
EVQLVQSGAEVKKPGESLRISCKGSGYTFTSYWMYWVRQAPGQGLEWMGRIDPNSGSTKYNEKFKNRVTISVDTSKNQFSLKLSSVTAADTAVYYCARDYRKGLYAMDYWGQG

SEQ ID NO: 255 - protein, 113 aa, synthetic construct
  REGION 1..113: note = source = /note="Description of Artificial Sequence: Synthetic polypeptide"
QVQLVQSGAEVKKPGASVKVSCKASGYTFTSYWMYWIRQSPSRGLEWLGRIDPNSGSTKYNEKFKNRFTISRDDSKNTAYLQMNSLKTEDTAVYYCARDYRKGLYAMDYWGQG

SEQ ID NO: 256 - protein, 113 aa, synthetic construct
  REGION 1..113: note = source = /note="Description of Artificial Sequence: Synthetic polypeptide"
EVQLVQSGAEVKKPGESLRISCKGSGYTFTSYWMYWVRQARGQRLEWIGRIDPNSGSTKYNEKFKNRLTISKDTSKNQVVLTMTNMDPVDTATYYCARDYRKGLYAMDYWGQG

SEQ ID NO: 257 - protein, 113 aa, synthetic construct
  REGION 1..113: note = source = /note="Description of Artificial Sequence: Synthetic polypeptide"
EVQLVQSGAEVKKPGATVKISCKVSGYTFTSYWMYWIRQSPSRGLEWLGRIDPNSGSTKYNEKFKNRLTISKDTSKNQVVLTMTNMDPVDTATYYCARDYRKGLYAMDYWGQG

SEQ ID NO: 258 - protein, 113 aa, synthetic construct
  REGION 1..113: note = source = /note="Description of Artificial Sequence: Synthetic polypeptide"
QITLKESGPTLVKPTQTLTLTCTFSGYTFTSYWMYWVRQAPGKGLEWVSRIDPNSGSTKYNEKFKNRVTITADKSTSTAYMELSSLRSEDTAVYYCARDYRKGLYAMDYWGQG

SEQ ID NO: 259 - protein, 113 aa, synthetic construct
  REGION 1..113: note = source = /note="Description of Artificial Sequence: Synthetic polypeptide"
EVQLVQSGAEVKKPGATVKISCKVSGYTFTSYWMYWVRQARGQRLEWIGRIDPNSGSTKYNEKFKNRFTISRDNSKNTLYLQMNSLRAEDTAVYYCARDYRKGLYAMDYWGQG

SEQ ID NO: 260 - protein, 446 aa, synthetic construct
  REGION 1..446: note = source = /note="Description of Artificial Sequence: Synthetic polypeptide"
EVQLVQSGAEVKKPGESLRISCKGSGYTFTSYWMYWIRQPPGKGLEWIGRIDPNSGSTKYNEKFKNRVTITADKSTSTAYMELSSLRSEDTAVYYCARDYRKGLYAMDYWGQGTTVTVSSASTKGPSVFPLAPCSRSTSESTAALGCLVKDYFPEPVTVSWNSGALTSGVHTFPAVLQSSGLYSLSSVVTVPSSSLGTKTYTCNVDHKPSNTKVDKRVESKYGPPCPPCPAPEFLGGPSVFLFPPKPKDTLMISRTPEVTCVVVDVSQEDPEVQFNWYVDGVEVHNAKTKPREEQFNSTYRVVSVLTVLHQDWLNGKEYKCKVSNKGLPSSIEKTISKAKGQPREPQVYTLPPSQEEMTKNQVSLTCLVKGFYPSDIAVEWESNGQPENNYKTTPPVLDSDGSFFLYSRLTVDKSRWQEGNVFSCSVMHEALHNHYTQKSLSLSLG

SEQ ID NO: 261 - protein, 7 aa, synthetic construct
  REGION 1..7: note = source = /note="Description of Artificial Sequence: Synthetic peptide"
GYTFTTY

SEQ ID NO: 262 - protein, 6 aa, synthetic construct
  REGION 1..6: note = source = /note="Description of Artificial Sequence: Synthetic peptide"
YPGTGG

SEQ ID NO: 263 - protein, 8 aa, synthetic construct
  REGION 1..8: note = source = /note="Description of Artificial Sequence: Synthetic peptide"
WTTGTGAY

SEQ ID NO: 264 - protein, 13 aa, synthetic construct
  REGION 1..13: note = source = /note="Description of Artificial Sequence: Synthetic peptide"
SQSLLDSGNQKNF

SEQ ID NO: 265 - skipped

SEQ ID NO: 266 - protein, 6 aa, synthetic construct
  REGION 1..6: note = source = /note="Description of Artificial Sequence: Synthetic peptide"
DYSYPY

SEQ ID NO: 267 - protein, 5 aa, synthetic construct
  REGION 1..5: note = source = /note="Description of Artificial Sequence: Synthetic peptide"
TYWMH

SEQ ID NO: 268 - protein, 17 aa, synthetic construct
  REGION 1..17: note = source = /note="Description of Artificial Sequence: Synthetic peptide"
NIYPGTGGSNFDEKFKN

SEQ ID NO: 269 - protein, 17 aa, synthetic construct
  REGION 1..17: note = source = /note="Description of Artificial Sequence: Synthetic peptide"
KSSQSLLDSGNQKNFLT

SEQ ID NO: 270 - protein, 7 aa, synthetic construct
  REGION 1..7: note = source = /note="Description of Artificial Sequence: Synthetic peptide"
WASTRES

SEQ ID NO: 271 - protein, 9 aa, synthetic construct
  REGION 1..9: note = source = /note="Description of Artificial Sequence: Synthetic peptide"
QNDYSYPYT

SEQ ID NO: 272 - protein, 10 aa, synthetic construct
  REGION 1..10: note = source = /note="Description of Artificial Sequence: Synthetic peptide"
GYTFTTYWMH

SEQ ID NO: 273 - protein, 5 aa, synthetic construct
  REGION 1..5: note = source = /note="Description of Artificial Sequence: Synthetic peptide"
NYGMN

SEQ ID NO: 274 - protein, 7 aa, synthetic construct
  REGION 1..7: note = source = /note="Description of Artificial Sequence: Synthetic peptide"
GFTLTNY

SEQ ID NO: 275 - protein, 10 aa, synthetic construct
  REGION 1..10: note = source = /note="Description of Artificial Sequence: Synthetic peptide"
GFTLTNYGMN

SEQ ID NO: 276 - protein, 17 aa, synthetic construct
  REGION 1..17: note = source = /note="Description of Artificial Sequence: Synthetic peptide"
WINTDTGEPTYADDFKG

SEQ ID NO: 277 - protein, 16 aa, synthetic construct
  REGION 1..16: note = source = /note="Description of Artificial Sequence: Synthetic peptide"
NPPYYYGTNNAEAMDY

SEQ ID NO: 278 - protein, 11 aa, synthetic construct
  REGION 1..11: note = source = /note="Description of Artificial Sequence: Synthetic peptide"
SSSQDISNYLN

SEQ ID NO: 279 - protein, 7 aa, synthetic construct
  REGION 1..7: note = source = /note="Description of Artificial Sequence: Synthetic peptide"
YTSTLHL

SEQ ID NO: 280 - protein, 9 aa, synthetic construct
  REGION 1..9: note = source = /note="Description of Artificial Sequence: Synthetic peptide"
QQYYNLPWT

SEQ ID NO: 281 - protein, 6 aa, synthetic construct
  REGION 1..6: note = source = /note="Description of Artificial Sequence: Synthetic peptide"
NTDTGE

SEQ ID NO: 282 - protein, 7 aa, synthetic construct
  REGION 1..7: note = source = /note="Description of Artificial Sequence: Synthetic peptide"
SQDISNY

SEQ ID NO: 283 - skipped

SEQ ID NO: 284 - protein, 6 aa, synthetic construct
  REGION 1..6: note = source = /note="Description of Artificial Sequence: Synthetic peptide"
YYNLPW

SEQ ID NO: 285 - protein, 7 aa, synthetic construct
  REGION 1..7: note = source = /note="Description of Artificial Sequence: Synthetic peptide"
GYTFTSY

SEQ ID NO: 286 - protein, 6 aa, synthetic construct
  REGION 1..6: note = source = /note="Description of Artificial Sequence: Synthetic peptide"
YPGNGD

SEQ ID NO: 287 - protein, 9 aa, synthetic construct
  REGION 1..9: note = source = /note="Description of Artificial Sequence: Synthetic peptide"
VGGAFPMDY

SEQ ID NO: 288 - protein, 11 aa, synthetic construct
  REGION 1..11: note = source = /note="Description of Artificial Sequence: Synthetic peptide"
SESVEYYGTSL

SEQ ID NO: 289 - skipped

SEQ ID NO: 290 - protein, 6 aa, synthetic construct
  REGION 1..6: note = source = /note="Description of Artificial Sequence: Synthetic peptide"
SRKDPS

SEQ ID NO: 291 - protein, 5 aa, synthetic construct
  REGION 1..5: note = source = /note="Description of Artificial Sequence: Synthetic peptide"
SYNMH

SEQ ID NO: 292 - protein, 17 aa, synthetic construct
  REGION 1..17: note = source = /note="Description of Artificial Sequence: Synthetic peptide"
DIYPGNGDTSYNQKFKG

SEQ ID NO: 293 - protein, 15 aa, synthetic construct
  REGION 1..15: note = source = /note="Description of Artificial Sequence: Synthetic peptide"
RASESVEYYGTSLMQ

SEQ ID NO: 294 - protein, 7 aa, synthetic construct
  REGION 1..7: note = source = /note="Description of Artificial Sequence: Synthetic peptide"
AASNVES

SEQ ID NO: 295 - protein, 9 aa, synthetic construct
  REGION 1..9: note = source = /note="Description of Artificial Sequence: Synthetic peptide"
QQSRKDPST

SEQ ID NO: 296 - protein, 6 aa, synthetic construct
  REGION 1..6: note = source = /note="Description of Artificial Sequence: Synthetic peptide"
YPGSGD

SEQ ID NO: 297 - protein, 17 aa, synthetic construct
  REGION 1..17: note = source = /note="Description of Artificial Sequence: Synthetic peptide"
DIYPGSGDTSYNQKFKG

SEQ ID NO: 298 - protein, 6 aa, synthetic construct
  REGION 1..6: note = source = /note="Description of Artificial Sequence: Synthetic peptide"
YPGQGD

SEQ ID NO: 299 - protein, 17 aa, synthetic construct
  REGION 1..17: note = source = /note="Description of Artificial Sequence: Synthetic peptide"
DIYPGQGDTSYNQKFKG

SEQ ID NO: 300 - protein, 447 aa, synthetic construct
  REGION 1..447: note = source = /note="Description of Artificial Sequence: Synthetic polypeptide"
QVQLVQSGAEVKKPGSSVKVSCKASGYTFSSNVISWVRQAPGQGLEWMGGVIPIVDIANYAQRFKGRVTITADESTSTTYMELSSLRSEDTAVYYCASTLGLVLDAMDYWGQGTLVTVSSASTKGPSVFPLAPCSRSTSESTAALGCLVKDYFPEPVTVSWNSGALTSGVHTFPAVLQSSGLYSLSSVVTVPSSSLGTKTYTCNVDHKPSNTKVDKRVESKYGPPCPSCPAPEFLGGPSVFLFPPKPKDTLMISRTPEVTCVVVDVSQEDPEVQFNWYVDGVEVHNAKTKPREEQFNSTYRVVSVLTVLHQDWLNGKEYKCKVSNKGLPSSIEKTISKAKGQPREPQVYTLPPSQEEMTKNQVSLTCLVKGFYPSDIAVEWESNGQPENNYKTTPPVLDSDGSFFLYSRLTVDKSRWQEGNVFSCSVMHEALHNHYTQKSLSLSLGK

SEQ ID NO: 301 - protein, 215 aa, synthetic construct
  REGION 1..215: note = source = /note="Description of Artificial Sequence: Synthetic polypeptide"
ETVLTQSPGTLSLSPGERATLSCRASQSLGSSYLAWYQQKPGQAPRLLIYGASSRAPGIPDRFSGSGSGTDFTLTISRLEPEDFAVYYCQQYADSPITFGQGTRLEIKRTVAAPSVFIFPPSDEQLKSGTASVVCLLNNFYPREAKVQWKVDNALQSGNSQESVTEQDSKDSTYSLSSTLTLSKADYEKHKVYACEVTHQGLSSPVTKSFNRGEC

SEQ ID NO: 302 - protein, 121 aa, synthetic construct
  REGION 1..121: note = source = /note="Description of Artificial Sequence: Synthetic polypeptide"
QVQLVQSGAEVKKPGSSVKVSCKASGGTFSSYAISWVRQAPGQGLEWMGGIIPIFGTANYAQKFQGRVTITADESTSTAYMELSSLRSEDTAVYYCARGLWEVRALPSVYWGQGTLVTVSS

SEQ ID NO: 303 - protein, 109 aa, synthetic construct
  REGION 1..109: note = source = /note="Description of Artificial Sequence: Synthetic polypeptide"
SYELTQPPSVSVAPGQTARITCGANDIGSKSVHWYQQKAGQAPVLVVSEDIIRPSGIPERISGSNSGNTATLTISRVEAGDEADYYCQVWDRDSDQYVFGTGTKVTVLG

SEQ ID NO: 304 - protein, 440 aa, synthetic construct
  REGION 1..440: note = source = /note="Description of Artificial Sequence: Synthetic polypeptide"
QVQLVESGGGVVQPGRSLRLDCKASGITFSNSGMHWVRQAPGKGLEWVAVIWYDGSKRYYADSVKGRFTISRDNSKNTLFLQMNSLRAEDTAVYYCATNDDYWGQGTLVTVSSASTKGPSVFPLAPCSRSTSESTAALGCLVKDYFPEPVTVSWNSGALTSGVHTFPAVLQSSGLYSLSSVVTVPSSSLGTKTYTCNVDHKPSNTKVDKRVESKYGPPCPPCPAPEFLGGPSVFLFPPKPKDTLMISRTPEVTCVVVDVSQEDPEVQFNWYVDGVEVHNAKTKPREEQFNSTYRVVSVLTVLHQDWLNGKEYKCKVSNKGLPSSIEKTISKAKGQPREPQVYTLPPSQEEMTKNQVSLTCLVKGFYPSDIAVEWESNGQPENNYKTTPPVLDSDGSFFLYSRLTVDKSRWQEGNVFSCSVMHEALHNHYTQKSLSLSLGK

SEQ ID NO: 305 - protein, 214 aa, synthetic construct
  REGION 1..214: note = source = /note="Description of Artificial Sequence: Synthetic polypeptide"
EIVLTQSPATLSLSPGERATLSCRASQSVSSYLAWYQQKPGQAPRLLIYDASNRATGIPARFSGSGSGTDFTLTISSLEPEDFAVYYCQQSSNWPRTFGQGTKVEIKRTVAAPSVFIFPPSDEQLKSGTASVVCLLNNFYPREAKVQWKVDNALQSGNSQESVTEQDSKDSTYSLSSTLTLSKADYEKHKVYACEVTHQGLSSPVTKSFNRGEC

SEQ ID NO: 306 - protein, 447 aa, synthetic construct
  REGION 1..447: note = source = /note="Description of Artificial Sequence: Synthetic polypeptide"
QVQLVQSGVEVKKPGASVKVSCKASGYTFTNYYMYWVRQAPGQGLEWMGGINPSNGGTNFNEKFKNRVTLTTDSSTTTAYMELKSLQFDDTAVYYCARRDYRFDMGFDYWGQGTTVTVSSASTKGPSVFPLAPCSRSTSESTAALGCLVKDYFPEPVTVSWNSGALTSGVHTFPAVLQSSGLYSLSSVVTVPSSSLGTKTYTCNVDHKPSNTKVDKRVESKYGPPCPPCPAPEFLGGPSVFLFPPKPKDTLMISRTPEVTCVVVDVSQEDPEVQFNWYVDGVEVHNAKTKPREEQFNSTYRVVSVLTVLHQDWLNGKEYKCKVSNKGLPSSIEKTISKAKGQPREPQVYTLPPSQEEMTKNQVSLTCLVKGFYPSDIAVEWESNGQPENNYKTTPPVLDSDGSFFLYSRLTVDKSRWQEGNVFSCSVMHEALHNHYTQKSLSLSLGK

SEQ ID NO: 307 - protein, 218 aa, synthetic construct
  REGION 1..218: note = source = /note="Description of Artificial Sequence: Synthetic polypeptide"
EIVLTQSPATLSLSPGERATLSCRASKGVSTSGYSYLHWYQQKPGQAPRLLIYLASYLESGVPARFSGSGSGTDFTLTISSLEPEDFAVYYCQHSRDLPLTFGGGTKVEIKRTVAAPSVFIFPPSDEQLKSGTASVVCLLNNFYPREAKVQWKVDNALQSGNSQESVTEQDSKDSTYSLSSTLTLSKADYEKHKVYACEVTHQGLSSPVTKSFNRGEC

SEQ ID NO: 308 - protein, 118 aa, synthetic construct
  REGION 1..118: note = source = /note="Description of Artificial Sequence: Synthetic polypeptide"
EVQLLESGGGLVQPGGSLRLSCAASGFTFSSYIMMWVRQAPGKGLEWVSSIYPSGGITFYADKGRFTISRDNSKNTLYLQMNSLRAEDTAVYYCARIKLGTVTTVDYWGQGTLVTVSS

SEQ ID NO: 309 - protein, 110 aa, synthetic construct
  REGION 1..110: note = source = /note="Description of Artificial Sequence: Synthetic polypeptide"
QSALTQPASVSGSPGQSITISCTGTSSDVGGYNYVSWYQQHPGKAPKLMIYDVSNRPSGVSNRFSGSKSGNTASLTISGLQAEDEADYYCSSYTSSSTRVFGTGTKVTVL

SEQ ID NO: 310 - protein, 253 aa, synthetic construct [sequence omitted]

SEQ ID NO: 311 - protein, 263 aa, synthetic construct [sequence omitted]

SEQ ID NO: 312 - protein, 117 aa, synthetic construct
  REGION 1..117: note = source = /note="Description of Artificial Sequence: Synthetic polypeptide"
EVQLLESGGGLVQPGGSLRLSCAASGFTFSSYAMSWVRQAPGKGLEWVSGIGSYGGGTYYADSVKGRFTISRDNSKNTLYLQMNSLRAEDTAVYYCARYVNFGMDYWGQGTLVTVSS

SEQ ID NO: 313 - protein, 107 aa, synthetic construct
  REGION 1..107: note = source = /note="Description of Artificial Sequence: Synthetic polypeptide"
DIQMTQSPSSLSASVGDRVTITCRASQSISSYLNWYQQKPGKAPKLLIYAASSLQSGVPSRFSGSGSGTDFTLTISSLQPEDFATYYCQQYGRNPPTFGQGTKLEIK

SEQ ID NO: 314 - protein, 8 aa, synthetic construct
  REGION 1..8: note = source = /note="Description of Artificial Sequence: Synthetic peptide"
GFTFSSYA

SEQ ID NO: 315 - protein, 8 aa, synthetic construct
  REGION 1..8: note = source = /note="Description of Artificial Sequence: Synthetic peptide"
IGSYGGGT

SEQ ID NO: 316 - protein, 10 aa, synthetic construct
  REGION 1..10: note = source = /note="Description of Artificial Sequence: Synthetic peptide"
ARYVNFGMDY

SEQ ID NO: 317 - protein, 6 aa, synthetic construct
  REGION 1..6: note = source = /note="Description of Artificial Sequence: Synthetic peptide"
QSISSY

SEQ ID NO: 318 - protein, 9 aa, synthetic construct
  REGION 1..9: note = source = /note="Description of Artificial Sequence: Synthetic peptide"
QQYGRNPPT

SEQ ID NO: 319 - protein, 116 aa, synthetic construct
  REGION 1..116: note = source = /note="Description of Artificial Sequence: Synthetic polypeptide"
EVQLLESGGGLVQPGGSLRLSCAASGFTFSSYAMSWVRQAPGKGLEWVSAISGSGGSTYYADSVKGRFTISRDNSKNTLYLQMNSLRAEDTAVYYCARRVWGFDYWGQGTLVTVSS

SEQ ID NO: 320 - protein, 107 aa, synthetic construct
  REGION 1..107: note = source = /note="Description of Artificial Sequence: Synthetic polypeptide"
DIQMTQSPSSLSASVGDRVTITCRASQSISSYLNWYQQKPGKAPKLLIYAASSLQSGVPSRFSGSGSGTDFTLTISSLQPEDFATYYCQQYGVYPFTFGQGTKLEIK

SEQ ID NO: 321 - protein, 8 aa, synthetic construct
  REGION 1..8: note = source = /note="Description of Artificial Sequence: Synthetic peptide"
ISGSGGST

SEQ ID NO: 322 - protein, 9 aa, synthetic construct
  REGION 1..9: note = source = /note="Description of Artificial Sequence: Synthetic peptide"
ARRVWGFDY

SEQ ID NO: 323 - protein, 9 aa, synthetic construct
  REGION 1..9: note = source = /note="Description of Artificial Sequence: Synthetic peptide"
QQYGVYPFT

SEQ ID NO: 324 - protein, 128 aa, synthetic construct
  MOD_RES 120: note = Any amino acid
  MOD_RES 124..125: note = Any amino acid
  REGION 1..128: note = source = /note="Description of Artificial Sequence: Synthetic polypeptide"
EVRLQQSGADLVKPGASVKLSCASGFIIKATYMHWVRQRPEQGLEWIGRIDPANGEKYDPKFQVKAITADTSSSTAYLQLNSLTSDDTAVYYCARYAWYFDVWGAGTTVTVSSAKTTPPXVYPXXPGS

SEQ ID NO: 325 - protein, 127 aa, synthetic construct
  REGION 1..127: note = source = /note="Description of Artificial Sequence: Synthetic polypeptide"
DIQMTQSPASLSASVGDTVTITCRASENIYSFLAWYHQKQGRSPQLLVYHAKTLAEGVPSRFSGSGSGTQFSLKINSLQAEDFGSYYCQHYYGSPLTFGAGTKLEVKRADAAPTVSIFPPSSEELSL

SEQ ID NO: 326 - protein, 10 aa, synthetic construct
  REGION 1..10: note = source = /note="Description of Artificial Sequence: Synthetic peptide"
GFIIKATYMH

SEQ ID NO: 327 - protein, 17 aa, synthetic construct
  REGION 1..17: note = source = /note="Description of Artificial Sequence: Synthetic peptide"
RIDPANGETKYDPKFQV

SEQ ID NO: 328 - protein, 7 aa, synthetic construct
  REGION 1..7: note = source = /note="Description of Artificial Sequence: Synthetic peptide"
YAWYFDV

SEQ ID NO: 329 - protein, 11 aa, synthetic construct
  REGION 1..11: note = source = /note="Description of Artificial Sequence: Synthetic peptide"
RASENIYSFLA

SEQ ID NO: 330 - protein, 7 aa, synthetic construct
  REGION 1..7: note = source = /note="Description of Artificial Sequence: Synthetic peptide"
HAKTLAE

SEQ ID NO: 331 - protein, 9 aa, synthetic construct
  REGION 1..9: note = source = /note="Description of Artificial Sequence: Synthetic peptide"
QHYYGSPLT

SEQ ID NO: 332 - protein, 127 aa, synthetic construct [sequence omitted]

SEQ ID NO: 333 - protein, 127 aa, synthetic construct [sequence omitted]

SEQ ID NO: 334 - protein, 5 aa, synthetic construct
  REGION 1..5: note = source = /note="Description of Artificial Sequence: Synthetic peptide"
NYWMN

SEQ ID NO: 335 - protein, 17 aa, synthetic construct
  REGION 1..17: note = source = /note="Description of Artificial Sequence: Synthetic peptide"
AINQDGSEKYYVGSVKG

SEQ ID NO: 336 - protein, 18 aa, synthetic construct
  REGION 1..18: note = source = /note="Description of Artificial Sequence: Synthetic peptide"
DYYDILTDYYIHYWYFDL

SEQ ID NO: 337 - protein, 12 aa, synthetic construct
  REGION 1..12: note = source = /note="Description of Artificial Sequence: Synthetic peptide"
RASQSVSSSYLA

SEQ ID NO: 338 - protein, 7 aa, synthetic construct
  REGION 1..7: note = source = /note="Description of Artificial Sequence: Synthetic peptide"
GASSRAT

SEQ ID NO: 339 - protein, 446 aa, synthetic construct
  REGION 1..446: note = source = /note="Description of Artificial Sequence: Synthetic polypeptide"
EVQLVESGGDLVQPGGSLRLSCAASGFTFSSYWMSWVRQAPGKGLEWVANIKQDGSEKYYVDSVKGRFTISRDNAKNSLYLQMNSLRAEDTAVYYCARDRGSLYYWGQGTLVTVSSASTKGPSVFPLAPSSKSTSGGTAALGCLVKDYFPEPVTVSWNSGALTSGVHTFPAVLQSSGLYSLSSVVTVPSSSLGTQTYICNVNHKPSNTKVDKRVEPKSCDKTHTCPPCPAPELLGGPSVFLFPPKPKDTLMISRTPEVTCVVVDVSHEDPEVKFNWYVDGVEVHNAKTKPREEQYNSTYRVVSVLTVLHQDWLNGKEYKCKVSNKALPAPIEKTISKAKGQPREPQVYTLPPSREEMTKNQVSLTCLVKGFYPSDIAVEWESNGQPENNYKTTPPVLDSDGSFFLYSKLTVDKSRWQQGNVFSCSVMHEALHNHYTQKSLSLSPGK

SEQ ID NO: 340 - protein, 214 aa, synthetic construct
  REGION 1..214: note = source = /note="Description of Artificial Sequence: Synthetic polypeptide"
AIQLTQSPSSLSASVGDRVTITCRPSQGINWELAWYQQKPGKAPKLLIYDASSLEQGVPSRFSGSGSGTDFTLTISSLQPEDFATYYCQQFNSYPLTFGGGTKVEIKRTVAAPSVFIFPPSDEQLKSGTASVVCLLNNFYPREAKVQWKVDNALQSGNSQESVTEQDSKDSTYSLSSTLTLSKADYEKHKVYACEVTHQGLSSPVTKSFNRGEC

SEQ ID NO: 341 - protein, 119 aa, synthetic construct
  REGION 1..119: note = source = /note="Description of Artificial Sequence: Synthetic polypeptide"
QVQLVQSGAEVKKPGSSVKVSCKASGYSFTDYHIHWVRQAPGQGLEWMGVINPMYGTTDYNQRFKGRVTITADESTSTAYMELSSLRSEDTAVYYCARYDYFTGTGVYWGQGTLVTVSS

SEQ ID NO: 342 - protein, 112 aa, synthetic construct
  REGION 1..112: note = source = /note="Description of Artificial Sequence: Synthetic polypeptide"
DIVMTQTPLSLSVTPGQPASISCRSSRSLVHSRGNTYLHWYLQKPGQSPQLLIYKVSNRFIGVPDRFSGSGSGTDFTLKISRVEAEDVGVYYCSQSTHLPFTFGQGTKLEIK

SEQ ID NO: 343 - protein, 5 aa, synthetic construct
  REGION 1..5: note = source = /note="Description of Artificial Sequence: Synthetic peptide"
RYGIS

SEQ ID NO: 344 - protein, 17 aa, synthetic construct
  REGION 1..17: note = source = /note="Description of Artificial Sequence: Synthetic peptide"
WISTYSGNTNYAQKLQG

SEQ ID NO: 345 - protein, 7 aa, synthetic construct
  REGION 1..7: note = source = /note="Description of Artificial Sequence: Synthetic peptide"
RQLYFDY

SEQ ID NO: 346 - protein, 11 aa, synthetic construct
  REGION 1..11: note = source = /note="Description of Artificial Sequence: Synthetic peptide"
RASQSVSSNLA

SEQ ID NO: 347 - protein, 7 aa, synthetic construct
  REGION 1..7: note = source = /note="Description of Artificial Sequence: Synthetic peptide"
DASTRAT

SEQ ID NO: 348 - protein, 9 aa, synthetic construct
  REGION 1..9: note = source = /note="Description of Artificial Sequence: Synthetic peptide"
QQYDNWPLT

SEQ ID NO: 349 - protein, 137 aa, synthetic construct
  REGION 1..137: note = source = /note="Description of Artificial Sequence: Synthetic polypeptide"
MEFGLSWVFLVALLRGVQCQVQLVESGGGVVQPGRSLRLSCAASGFTFSVYGMNWVRQAPGKGLEWVAIIWYDGDNQYYADSVKGRFTISRDNSKNTLYLQMNGLRAEDTAVYYCARDLRTGPFDYWGQGTLVTVSS

SEQ ID NO: 350 - protein, 126 aa, synthetic construct
  REGION 1..126: note = source = /note="Description of Artificial Sequence: Synthetic polypeptide"
MLPSQLIGFLLLWVPASRGEIVLTQSPDFQSVTPKEKVTITCRASQSIGSSLHWYQQKPDQSPKLLIKYASQSFSGVPSRFSGSGSGTDFTLTINSLEAEDAAAYYCHQSSSLPFTFGPGTKVDIK

SEQ ID NO: 351 - protein, 12 aa, synthetic construct
  REGION 1..12: note = source = /note="Description of Artificial Sequence: Synthetic peptide"
GDSVSSNSAAWG

SEQ ID NO: 352 - protein, 18 aa, synthetic construct
  REGION 1..18: note = source = /note="Description of Artificial Sequence: Synthetic peptide"
RIYYRSKWYNSYAVSVKS

SEQ ID NO: 353 - protein, 12 aa, synthetic construct
  REGION 1..12: note = source = /note="Description of Artificial Sequence: Synthetic peptide"
RASQFISSSYLS

SEQ ID NO: 354 - protein, 11 aa, synthetic construct
  REGION 1..11: note = source = /note="Description of Artificial Sequence: Synthetic peptide"
LLIYGSSSRAT

SEQ ID NO: 355 - protein, 8 aa, synthetic construct
  REGION 1..8: note = source = /note="Description of Artificial Sequence: Synthetic peptide"
QQLYSSPM

SEQ ID NO: 356 - protein, 124 aa, synthetic construct
  REGION 1..124: note = source = /note="Description of Artificial Sequence: Synthetic polypeptide"
QVQLQQSGPGLVKPSQTLSLTCAISGDSVSSNSAAWGWIRQSPGRGLEWLGRIYYRSKWYNSYAVSVKSRITINPDTSKNQFSLQLNSVTPEDTAVYYCARYDWVPKIGVFDSWGQGTLVTVSS

SEQ ID NO: 357 - protein, 110 aa, synthetic construct
  REGION 1..110: note = source = /note="Description of Artificial Sequence: Synthetic polypeptide"
DIVLTQSPATLSLSPGERATLSCRASQFISSSYLSWYQQKPGQAPRLLIYGSSSRATGVPARFSGSGSGTDFTLTISSLEPEDFAVYYCQQLYSSPMTFGQGTKVEIKRT

SEQ ID NO: 358 - protein, 454 aa, synthetic construct
  REGION 1..454: note = source = /note="Description of Artificial Sequence: Synthetic polypeptide"
QVQLQQSGPGLVKPSQTLSLTCAISGDSVSSNSAAWGWIRQSPGRGLEWLGRIYYRSKWYNSYAVSVKSRITINPDTSKNQFSLQLNSVTPEDTAVYYCARYDWVPKIGVFDSWGQGTLVTVSSASTKGPSVFPLAPSSKSTSGGTAALGCLVKDYFPEPVTVSWNSGALTSGVHTFPAVLQSSGLYSLSSVVTVPSSSLGTQTYICNVNHKPSNTKVDKRVEPKSCDKTHTCPPCPAPELLGGPSVFLFPPKPKDTLMISRTPEVTCVVVDVSHEDPEVKFNWYVDGVEVHNAKTKPREEQYNSTYRVVSVLTVLHQDWLNGKEYKCKVSNKALPAPIEKTISKAKGQPREPQVYTLPPSREEMTKNQVSLTCLVKGFYPSDIAVEWESNGQPENNYKTTPPVLDSDGSFFLYSKLTVDKSRWQQGNVFSCSVMHEALHNHYTQKSLSLSPGK

SEQ ID NO: 359 - protein, 215 aa, synthetic construct
  REGION 1..215: note = source = /note="Description of Artificial Sequence: Synthetic polypeptide"
DIVLTQSPATLSLSPGERATLSCRASQFISSSYLSWYQQKPGQAPRLLIYGSSSRATGVPARFSGSGSGTDFTLTISSLEPEDFAVYYCQQLYSSPMTFGQGTKVEIKRTVAAPSVFIFPPSDEQLKSGTASVVCLLNNFYPREAKVQWKVDNALQSGNSQESVTEQDSKDSTYSLSSTLTLSKADYEKHKVYACEVTHQGLSSPVTKSFNRGEC

SEQ ID NO: 360 - protein, 4 aa, synthetic construct
  REGION 1..4: note = source = /note="Description of Artificial Sequence: Synthetic peptide"
RGDS

SEQ ID NO: 361 - protein, 9 aa, synthetic construct
  REGION 1..9: note = source = /note="Description of Artificial Sequence: Synthetic peptide"
QQYGSSPCT

SEQ ID NO: 362 - protein, 12 aa, synthetic construct
  REGION 1..12: note = source = /note="Description of Artificial Sequence: Synthetic peptide"
YDWVPKIGVFDS